European Patent Specification EP 3 439 682 B1, published August 13, 2025. Title: HYPERSENSITIVE RESPONSE ELICITOR-DERIVED PEPTIDES AND USE THEREOF. Applicant: PLANT HEALTH CARE, INC. The sequence listing filed with the application follows.

SEQUENCE LISTING (549 sequences)

SEQ ID NO: 1 - protein, 13 aa, Artificial
  Consensus peptide
  MISC_FEATURE (1)..(1): X at position 1 is L, I, V, or F
  MISC_FEATURE (2)..(2): X at position 2 is any amino acid
  MISC_FEATURE (3)..(3): X at position 3 is optional, any amino acid
  MISC_FEATURE (4)..(4): X at position 4 is L, I, V, or F
  MISC_FEATURE (5)..(5): X at position 5 is L, I, V, or F
  MISC_FEATURE (6)..(6): X at position 6 is L, I, V, or F
  MISC_FEATURE (7)..(7): X at position 7 is any amino acid
  MISC_FEATURE (8)..(8): X at position 8 is L, I, V or F
  MISC_FEATURE (9)..(9): X at position 9 is L, I, V or F
  MISC_FEATURE (10)..(10): X at position 10 is any amino acid
  MISC_FEATURE (11)..(11): X at position 11 is any amino acid
  MISC_FEATURE (12)..(12): X at position 12 is any amino acid
  MISC_FEATURE (13)..(13): X at position 13 is L, I, V, or F
XXXXXXXXXXXXX

SEQ ID NO: 2 - protein, 13 aa, Artificial
  P5 consensus peptide
  MISC_FEATURE (2)..(2): X at position 2 is any amino acid
  MISC_FEATURE (3)..(3): X at position 3 is optional, any amino acid
  MISC_FEATURE (7)..(7): X at position 7 is any amino acid
  MISC_FEATURE (8)..(8): X at position 8 is F or L
  MISC_FEATURE (9)..(9): X at position 9 is I or L
  MISC_FEATURE (10)..(10): X at position 10 is any amino acid
  MISC_FEATURE (11)..(11): X at position 11 is any amino acid
  MISC_FEATURE (12)..(12): X at position 12 is any amino acid
LXXLLLXXXXXXL

SEQ ID NO: 3 - protein, 17 aa, Artificial
  Consensus peptide
  MISC_FEATURE (1)..(1): X at position 1 is Q or E
  MISC_FEATURE (2)..(2): X at position 2 is Q or E
  MISC_FEATURE (3)..(3): X at position 3 is L, I, V, or F
  MISC_FEATURE (4)..(4): X at position 4 is any amino acid
  MISC_FEATURE (5)..(5): X at position 5 is optional, any amino acid
  MISC_FEATURE (6)..(6): X at position 6 is L, I, V, or F
  MISC_FEATURE (7)..(7): X at position 7 is L, I, V, or F
  MISC_FEATURE (8)..(8): X at position 8 is L, I, V, or F
  MISC_FEATURE (9)..(9): X at position 9 is any amino acid
  MISC_FEATURE (10)..(10): X at position 10 is L, I, V, or F
  MISC_FEATURE (11)..(11): X at position 11 is L, I, V, or F
  MISC_FEATURE (12)..(12): X at position 12 is any amino acid
  MISC_FEATURE (13)..(13): X at position 13 is any amino acid
  MISC_FEATURE (14)..(14): X at position 14 is any amino acid
  MISC_FEATURE (15)..(15): X at position 15 is L, I, V, or F
  MISC_FEATURE (16)..(16): X at position 16 is D, G, Q, or E
  MISC_FEATURE (17)..(17): X at position 17 is D, G, Q, or E
XXXXXXXXXXXXXXXXX

SEQ ID NO: 4 - protein, 15 aa, Artificial
  Synthetic peptide
  MISC_FEATURE (1)..(1): X at position 1 is L, I, V, or F
  MISC_FEATURE (2)..(2): X at position 2 is any amino acid
  MISC_FEATURE (3)..(3): X at position 3 is optional, any amino acid
  MISC_FEATURE (4)..(4): X at position 4 is L, I, V, or F
  MISC_FEATURE (5)..(5): X at position 5 is L, I, V, or F
  MISC_FEATURE (6)..(6): X at position 6 is L, I, V, or F
  MISC_FEATURE (7)..(7): X at position 7 is any amino acid
  MISC_FEATURE (8)..(8): X at position 8 is L, I, V, or F
  MISC_FEATURE (9)..(9): X at position 9 is L, I, V, or F
  MISC_FEATURE (10)..(10): X at position 10 is any amino acid
  MISC_FEATURE (11)..(11): X at position 11 is any amino acid
  MISC_FEATURE (12)..(12): X at position 12 is any amino acid
  MISC_FEATURE (13)..(13): X at position 13 is L, I, V, or F
  MISC_FEATURE (14)..(14): X at position 14 is D, G, Q, or E
  MISC_FEATURE (15)..(15): X at position 15 is D, G, Q, or E
XXXXXXXXXXXXXXX

SEQ ID NO: 5 - protein, 15 aa, Artificial
  Synthetic peptide
  MISC_FEATURE (1)..(1): X at position 1 is Q or E
  MISC_FEATURE (2)..(2): X at position 2 is Q or E
  MISC_FEATURE (3)..(3): X at position 3 is L, I, V, or F
  MISC_FEATURE (4)..(4): X at position 4 is any amino acid
  MISC_FEATURE (5)..(5): X at position 5 is optional, any amino acid
  MISC_FEATURE (6)..(6): X at position 6 is L, I, V, or F
  MISC_FEATURE (7)..(7): X at position 7 is L, I, V, or F
  MISC_FEATURE (8)..(8): X at position 8 is L, I, V, or F
  MISC_FEATURE (9)..(9): X at position 9 is any amino acid
  MISC_FEATURE (10)..(10): X at position 10 is L, I, V, or F
  MISC_FEATURE (11)..(11): X at position 11 is L, I, V, or F
  MISC_FEATURE (12)..(12): X at position 12 is any amino acid
  MISC_FEATURE (13)..(13): X at position 13 is any amino acid
  MISC_FEATURE (14)..(14): X at position 14 is any amino acid
  MISC_FEATURE (15)..(15): X at position 15 is L, I, V, or F
XXXXXXXXXXXXXXX

SEQ ID NO: 6 - protein, 13 aa, Artificial
  Synthetic peptide
  MISC_FEATURE (1)..(1): X at position 1 is L, I, V, F, A, or a non-hydrophobic amino acid
  MISC_FEATURE (2)..(2): X at position 2 is any amino acid
  MISC_FEATURE (3)..(3): X at position 3 is optional, any amino acid
  MISC_FEATURE (4)..(4): X at position 4 is L, I, V, F, A, or a non-hydrophobic amino acid
  MISC_FEATURE (5)..(5): X at position 5 is L, I, V, F, A, or a non-hydrophobic amino acid
  MISC_FEATURE (6)..(6): X at position 6 is L, I, V, F, A, or a non-hydrophobic amino acid
  MISC_FEATURE (7)..(7): X at position 7 is any amino acid
  MISC_FEATURE (8)..(8): X at position 8 is L, I, V, F, A, or a non-hydrophobic amino acid
  MISC_FEATURE (9)..(9): X at position 9 is L, I, V, F, A, or a non-hydrophobic amino acid
  MISC_FEATURE (10)..(10): X at position 10 is any amino acid
  MISC_FEATURE (11)..(11): X at position 11 is any amino acid
  MISC_FEATURE (12)..(12): X at position 12 is any amino acid
  MISC_FEATURE (13)..(13): X at position 13 is L, I, V, F, A, or a non-hydrophobic amino acid
XXXXXXXXXXXXX

SEQ ID NO: 7 - protein, 22 aa, Artificial
  Wildtype peptide
SAGSEQQLDQLLAMFIMMMLQQ

SEQ ID NO: 8 - protein, 21 aa, Artificial
  Synthetic peptide
SAGSEQQLDLLLMFIMMMLQQ

SEQ ID NO: 9 - protein, 22 aa, Artificial
  Synthetic peptide
SAGSEQQLDQLLLMFIMMMLQQ

SEQ ID NO: 10 - protein, 21 aa, Artificial
  Synthetic peptide
SAGSEQQLDLLLMFIAAALQQ

SEQ ID NO: 11 - protein, 21 aa, Artificial
  Synthetic peptide
SAGSEQQLDLLLAFIAAALQQ

SEQ ID NO: 12 - protein, 21 aa, Artificial
  Synthetic peptide
SAGSEQQLELLLAFIAAALQQ

SEQ ID NO: 13 - protein, 18 aa, Artificial
  Synthetic peptide
SEEEEELDLLLAFIAAAL

SEQ ID NO: 14 - protein, 20 aa, Artificial
  Synthetic peptide
SEEEEELDLLLAFIAAALQQ

SEQ ID NO: 15 - protein, 18 aa, Artificial
  Synthetic peptide
LDLLLAFIAAALEEEEEE

SEQ ID NO: 16 - protein, 16 aa, Artificial
  Synthetic peptide
LDLLLAFIEEELEEEE

SEQ ID NO: 17 - protein, 18 aa, Artificial
  Synthetic peptide
SEEELDLLLAFIAAALEE

SEQ ID NO: 18 - protein, 18 aa, Artificial
  Synthetic peptide
SEEELDLLLAFIEEELEE

SEQ ID NO: 19 - protein, 18 aa, Artificial
  Synthetic peptide
SEEELDLLLAFIAAALDD

SEQ ID NO: 20 - protein, 20 aa, Artificial
  Synthetic peptide
SEEEEELDLLLAFIAAALGG

SEQ ID NO: 21 - protein, 22 aa, Artificial
  Synthetic peptide
SEEEEEEELDLLLAFIAAALAA

SEQ ID NO: 22 - protein, 21 aa, Artificial
  Synthetic peptide
SEEEEEELDLLLAFIAAALSS

SEQ ID NO: 23 - protein, 21 aa, Artificial
  Synthetic peptide
SAGSEQQLDLLLGFIGGGLQQ

SEQ ID NO: 24 - protein, 21 aa, Artificial
  Synthetic peptide
SAGSEQQLDLLLSFISSSLQQ

SEQ ID NO: 25 - protein, 19 aa, Artificial
  Synthetic peptide
SEEEEELDLLLAFIAAALQ

SEQ ID NO: 26 - protein, 19 aa, Artificial
  Synthetic peptide
SEEEEELDLLLAFIAAALS

SEQ ID NO: 27 - protein, 19 aa, Artificial
  Synthetic peptide
SEEEEELDLLLAFIAAALA

SEQ ID NO: 28 - protein, 19 aa, Artificial
  Synthetic peptide
SEEEEELDLLLAFIAAALE

SEQ ID NO: 29 - protein, 19 aa, Artificial
  Synthetic peptide
SELELLLAFIAAALEEEEE

SEQ ID NO: 30 - protein, 20 aa, Artificial
  Synthetic peptide
SEEELELLLAFIAAALEEEE

SEQ ID NO: 31 - protein, 19 aa, Artificial
  Synthetic peptide
SELDLLLAFIAAALEEEEE

SEQ ID NO: 32 - protein, 20 aa, Artificial
  Synthetic peptide
SEEEEELDLLLALIAAALQQ

SEQ ID NO: 33 - protein, 20 aa, Artificial
  Synthetic peptide
SEEQLELLLAFIAAALQQEE

SEQ ID NO: 34 - protein, 19 aa, Artificial
  Synthetic peptide
SEEQLDLLLAFIAAALQEE

SEQ ID NO: 35 - protein, 16 aa, Artificial
  Synthetic peptide
SELELLLAFIEEELEE

SEQ ID NO: 36 - protein, 16 aa, Artificial
  Synthetic peptide
SELELLLEFIEEELEE

SEQ ID NO: 37 - protein, 15 aa, Artificial
  Synthetic peptide
SELELLLEFIEEELE

SEQ ID NO: 38 - protein, 15 aa, Artificial
  Synthetic peptide
SELELLLELIEEELE

SEQ ID NO: 39 - protein, 20 aa, Artificial
  Synthetic peptide
SEEQLDLLLEFIEEELQQEE

SEQ ID NO: 40 - protein, 19 aa, Artificial
  Synthetic peptide
SELDLLLAFIDDDLEEEEE

SEQ ID NO: 41 - protein, 21 aa, Artificial
  Synthetic peptide
SAGSEEELDLLLMFIMMMLEE

SEQ ID NO: 42 - protein, 18 aa, Artificial
  Synthetic peptide
SEEELDLLLMFIMMMLEE

SEQ ID NO: 43 - protein, 19 aa, Artificial
  Synthetic peptide
SEEEQLDLLLMFIMMMLEE

SEQ ID NO: 44 - protein, 20 aa, Artificial
  Synthetic peptide
SEEEQLDLLLMFIMMMLQEE

SEQ ID NO: 45 - protein, 20 aa, Artificial
  Synthetic peptide
SEEQLDLLLMFIMMMLQQEE

SEQ ID NO: 46 - protein, 13 aa, Artificial
  Synthetic peptide
LELLLEFIEEELE

SEQ ID NO: 47 - protein, 14 aa, Artificial
  Synthetic peptide
LELLLEFIEEELEE

SEQ ID NO: 48 - protein, 14 aa, Artificial
  Synthetic peptide
SELELLLEFIEEEL

SEQ ID NO: 49 - protein, 15 aa, Artificial
  Synthetic peptide
LDQLLLMFIMMMLQQ

SEQ ID NO: 50 - protein, 21 aa, Artificial
  Synthetic peptide
SEEEEELDQLLLAFIAAALQQ

SEQ ID NO: 51 - protein, 19 aa, Artificial
  Synthetic peptide
SEEEEELDQLLLAFIAAAL

SEQ ID NO: 52 - protein, 21 aa, Artificial
  Synthetic peptide
SEEEEQLDQLLLAFIAAALQQ

SEQ ID NO: 53 - protein, 20 aa, Artificial
  Synthetic peptide
SEEQLDQLLLAFIAAALQEE

SEQ ID NO: 54 - protein, 19 aa, Artificial
  Synthetic peptide
SEEQLDQLLLAFIAAALEE

SEQ ID NO: 55 - protein, 19 aa, Artificial
  Synthetic peptide
SEEELDQLLLMFIMMMLEE

SEQ ID NO: 56 - protein, 20 aa, Artificial
  Synthetic peptide
SEEEQLDQLLLMFIMMMLEE

SEQ ID NO: 57 - protein, 21 aa, Artificial
  Synthetic peptide
SEEEQLDQLLLMFIMMMLQEE

SEQ ID NO: 58 - protein, 21 aa, Artificial
  Synthetic peptide
SEEQLDQLLLMFIMMMLQQEE

SEQ ID NO: 59 - protein, 15 aa, Artificial
  Synthetic peptide
LDQLLLAFIAAALQQ

SEQ ID NO: 60 - protein, 15 aa, Artificial
  Synthetic peptide
LDQLLLEFIEEELQQ

SEQ ID NO: 61 - protein, 16 aa, Artificial
  Synthetic peptide
QLDQLLLMFIMMMLQQ

SEQ ID NO: 62 - protein, 16 aa, Artificial
  Synthetic peptide
QLDQLLLAFIAAALQQ

SEQ ID NO: 63 - protein, 16 aa, Artificial
  Synthetic peptide
QLDQLLLEFIEEELQQ

SEQ ID NO: 64 - protein, 17 aa, Artificial
  Synthetic peptide
QQLDQLLLMFIMMMLQQ

SEQ ID NO: 65 - protein, 17 aa, Artificial
  Synthetic peptide
QQLDQLLLAFIAAALQQ

SEQ ID NO: 66 - protein, 17 aa, Artificial
  Synthetic peptide
QQLDQLLLEFIEEELQQ

SEQ ID NO: 67 - protein, 13 aa, Artificial
  Synthetic peptide
LDQLLLMFIMMML

SEQ ID NO: 68 - protein, 13 aa, Artificial
  Synthetic peptide
LDQLLLAFIAAAL

SEQ ID NO: 69 - protein, 13 aa, Artificial
  Synthetic peptide
LDQLLLEFIEEEL

SEQ ID NO: 70 - protein, 22 aa, Artificial
  Synthetic peptide
SAGSEEELDQLLLMFIMMMLEE

SEQ ID NO: 71 - protein, 21 aa, Artificial
  Synthetic peptide
SAGSEQQEDLLLMFIMMMLQQ

SEQ ID NO: 72 - protein, 21 aa, Artificial
  Synthetic peptide
SAGSEQQLDELLMFIMMMLQQ

SEQ ID NO: 73 - protein, 21 aa, Artificial
  Synthetic peptide
SAGSEQQLDLELMFIMMMLQQ

SEQ ID NO: 74 - protein, 21 aa, Artificial
  Synthetic peptide
SAGSEQQLDLLEMFIMMMLQQ

SEQ ID NO: 75 - protein, 21 aa, Artificial
  Synthetic peptide
SAGSEQQLDLLLEFIMMMLQQ

SEQ ID NO: 76 - protein, 21 aa, Artificial
  Synthetic peptide
SAGSEQQLDLLLMEIMMMLQQ

SEQ ID NO: 77 - protein, 21 aa, Artificial
  Synthetic peptide
SAGSEQQLDLLLMFEMMMLQQ

SEQ ID NO: 78 - protein, 21 aa, Artificial
  Synthetic peptide
SAGSEQQLDLLLMFIEMMLQQ

SEQ ID NO: 79 - protein, 21 aa, Artificial
  Synthetic peptide
SAGSEQQLDLLLMFIMEMLQQ

SEQ ID NO: 80 - protein, 21 aa, Artificial
  Synthetic peptide
SAGSEQQLDLLLMFIMMELQQ

SEQ ID NO: 81 - protein, 21 aa, Artificial
  Synthetic peptide
SAGSEQQLDLLLMFIMMMEQQ

SEQ ID NO: 82 - protein, 21 aa, Artificial
  Synthetic peptide
SAGSEQQLKLLLMFIMMMLQQ

SEQ ID NO: 83 - protein, 21 aa, Artificial
  Synthetic peptide
SAGSESSLDLLLMFIMMMLQQ

SEQ ID NO: 84 - protein, 21 aa, Artificial
  Synthetic peptide
SAGSEQQLDLLLMFIMMMLSS

SEQ ID NO: 85 - protein, 21 aa, Artificial
  Synthetic peptide
SAGSEGGLDLLLMFIMMMLQQ

SEQ ID NO: 86 - protein, 21 aa, Artificial
  Synthetic peptide
SAGSEQQLDLLLMFIMMMLGG

SEQ ID NO: 87 - protein, 21 aa, Artificial
  Synthetic peptide
SAGSEQQVDLLLMFIMMMLQQ

SEQ ID NO: 88 - protein, 21 aa, Artificial
  Synthetic peptide
SAGSEQQLDVLLMFIMMMLQQ

SEQ ID NO: 89 - protein, 21 aa, Artificial
  Synthetic peptide
SAGSEQQLDLVLMFIMMMLQQ

SEQ ID NO: 90 - protein, 21 aa, Artificial
  Synthetic peptide
SAGSEQQLDLLVMFIMMMLQQ

SEQ ID NO: 91 - protein, 21 aa, Artificial
  Synthetic peptide
SAGSEQQLDLLLVFIMMMLQQ

SEQ ID NO: 92 - protein, 21 aa, Artificial
  Synthetic peptide
SAGSEQQLDLLLMVIMMMLQQ

SEQ ID NO: 93 - protein, 21 aa, Artificial
  Synthetic peptide
SAGSEQQLDLLLMFVMMMLQQ

SEQ ID NO: 94 - protein, 21 aa, Artificial
  Synthetic peptide
SAGSEQQLDLLLMFIVMMLQQ

SEQ ID NO: 95 - protein, 21 aa, Artificial
  Synthetic peptide
SAGSEQQLDLLLMFIMVMLQQ

SEQ ID NO: 96 - protein, 21 aa, Artificial
  Synthetic peptide
SAGSEQQLDLLLMFIMMVLQQ

SEQ ID NO: 97 - protein, 21 aa, Artificial
  Synthetic peptide
SAGSEQQLDLLLMFIMMMVQQ

SEQ ID NO: 98 - protein, 22 aa, Artificial
  Synthetic peptide
SAGSEQQEDQLLLMFIMMMLQQ

SEQ ID NO: 99 - protein, 22 aa, Artificial
  Synthetic peptide
SAGSEQQLDQELLMFIMMMLQQ

SEQ ID NO: 100 - protein, 22 aa, Artificial
  Synthetic peptide
SAGSEQQLDQLELMFIMMMLQQ

SEQ ID NO: 101 - protein, 22 aa, Artificial
  Synthetic peptide
SAGSEQQLDQLLEMFIMMMLQQ

SEQ ID NO: 102 - protein, 22 aa, Artificial
  Synthetic peptide
SAGSEQQLDQLLLEFIMMMLQQ

SEQ ID NO: 103 - protein, 22 aa, Artificial
  Synthetic peptide
SAGSEQQLDQLLLMEIMMMLQQ

SEQ ID NO: 104 - protein, 22 aa, Artificial
  Synthetic peptide
SAGSEQQLDQLLLMFEMMMLQQ

SEQ ID NO: 105 - protein, 22 aa, Artificial
  Synthetic peptide
SAGSEQQLDQLLLMFIEMMLQQ

SEQ ID NO: 106 - protein, 22 aa, Artificial
  Synthetic peptide
SAGSEQQLDQLLLMFIMEMLQQ

SEQ ID NO: 107 - protein, 22 aa, Artificial
  Synthetic peptide
SAGSEQQLDQLLLMFIMMELQQ

SEQ ID NO: 108 - protein, 22 aa, Artificial
  Synthetic peptide
SAGSEQQLDQLLLMFIMMMEQQ

SEQ ID NO: 109 - protein, 22 aa, Artificial
  Synthetic peptide
SAGSEQQLKQLLLMFIMMMLQQ

SEQ ID NO: 110 - protein, 22 aa, Artificial
  Synthetic peptide
SAGSEQQLDELLLMFIMMMLQQ

SEQ ID NO: 111 - protein, 22 aa, Artificial
  Synthetic peptide
SAGSEQQLDSLLLMFIMMMLQQ

SEQ ID NO: 112 - protein, 22 aa, Artificial
  Synthetic peptide
SAGSEQQLDALLLMFIMMMLQQ

SEQ ID NO: 113 - protein, 22 aa, Artificial
  Synthetic peptide
SAGSESSLDQLLLMFIMMMLQQ

SEQ ID NO: 114 - protein, 22 aa, Artificial
  Synthetic peptide
SAGSEQQLDQLLLMFIMMMLSS

SEQ ID NO: 115 - protein, 22 aa, Artificial
  Synthetic peptide
SAGSEGGLDQLLLMFIMMMLQQ

SEQ ID NO: 116 - protein, 22 aa, Artificial
  Synthetic peptide
SAGSEQQLDQLLLMFIMMMLGG

SEQ ID NO: 117 - protein, 22 aa, Artificial
  Synthetic peptide
SAGSEQQVDQLLLMFIMMMLQQ

SEQ ID NO: 118 - protein, 22 aa, Artificial
  Synthetic peptide
SAGSEQQLDQVLLMFIMMMLQQ

SEQ ID NO: 119 - protein, 22 aa, Artificial
  Synthetic peptide
SAGSEQQLDQLVLMFIMMMLQQ

SEQ ID NO: 120 - protein, 22 aa, Artificial
  Synthetic peptide
SAGSEQQLDQLLVMFIMMMLQQ

SEQ ID NO: 121 - protein, 22 aa, Artificial
  Synthetic peptide
SAGSEQQLDQLLLVFIMMMLQQ

SEQ ID NO: 122 - protein, 22 aa, Artificial
  Synthetic peptide
SAGSEQQLDQLLLMVIMMMLQQ

SEQ ID NO: 123 - protein, 22 aa, Artificial
  Synthetic peptide
SAGSEQQLDQLLLMFVMMMLQQ

SEQ ID NO: 124 - protein, 22 aa, Artificial
  Synthetic peptide
SAGSEQQLDQLLLMFIVMMLQQ

SEQ ID NO: 125 - protein, 22 aa, Artificial
  Synthetic peptide
SAGSEQQLDQLLLMFIMVMLQQ

SEQ ID NO: 126 - protein, 22 aa, Artificial
  Synthetic peptide
SAGSEQQLDQLLLMFIMMVLQQ

SEQ ID NO: 127 - protein, 22 aa, Artificial
  Synthetic peptide
SAGSEQQLDQLLLMFIMMMVQQ

SEQ ID NO: 128 - protein, 20 aa, Artificial
  Synthetic peptide
SAGSEQQLDQLLLMFIMMML

SEQ ID NO: 129 - protein, 15 aa, Artificial
  Synthetic peptide
QQLDQLLLMFIMMML

SEQ ID NO: 130 - protein, 22 aa, Artificial
  Synthetic peptide
SAGSEQQLDQLLLAFIAAALQQ

SEQ ID NO: 131 - protein, 22 aa, Artificial
  Synthetic peptide
SAGSEQQLDQLLLEFIEEELQQ

SEQ ID NO: 132 - protein, 16 aa, Artificial
  Synthetic peptide
QQLDLLLMFIMMMLQQ

SEQ ID NO: 133 - protein, 14 aa, Artificial
  Synthetic peptide
LDLLLMFIMMMLQQ

SEQ ID NO: 134 - protein, 19 aa, Artificial
  Synthetic peptide
SAGSEQQLDLLLMFIMMML

SEQ ID NO: 135 - protein, 15 aa, Artificial
  Synthetic peptide
QQLDLLLMFIIMMML

SEQ ID NO: 136 - protein, 12 aa, Artificial
  Synthetic peptide
LDLLLMFIMMML

SEQ ID NO: 137 - protein, 21 aa, Artificial
  Synthetic peptide
SAGSEQQLDLLLEFIEEELQQ

SEQ ID NO: 138 - protein, 23 aa, Artificial
  Synthetic peptide
HHHHHHRQQLDLLLAFIAAALQQ

SEQ ID NO: 139 - protein, 15 aa, Artificial
  Synthetic peptide
QLELLLAFIAAALQQ

SEQ ID NO: 140 - protein, 19 aa, Artificial
  Synthetic peptide
SAGSEQQLDLLLAFIAAAL

SEQ ID NO: 141 - protein, 12 aa, Artificial
  Synthetic peptide
  MISC_FEATURE (6)..(6): X at position 6 is A or E
LDLLLXFIMMML

SEQ ID NO: 142 - protein, 12 aa, Artificial
  Synthetic peptide
  MISC_FEATURE (9)..(9): X at position 9 is A or E
LDLLLMFIXMML

SEQ ID NO: 143 - protein, 12 aa, Artificial
  Synthetic peptide
  MISC_FEATURE (10)..(10): X at position 10 is A or E
LDLLLMFIMXML

SEQ ID NO: 144 - protein, 12 aa, Artificial
  Synthetic peptide
  MISC_FEATURE (11)..(11): X at position 11 is A or E
LDLLLMFIMMXL

SEQ ID NO: 145 - protein, 12 aa, Artificial
  Synthetic peptide
  MISC_FEATURE (6)..(6): X at position 6 is A or E
  MISC_FEATURE (9)..(9): X at position 9 is A or E
LDLLLXFIXMML

SEQ ID NO: 146 - protein, 12 aa, Artificial
  Synthetic peptide
  MISC_FEATURE (6)..(6): X at position 6 is A or E
  MISC_FEATURE (10)..(10): X at position 10 is A or E
LDLLLXFIMXML

SEQ ID NO: 147 - protein, 12 aa, Artificial
  Synthetic peptide
  MISC_FEATURE (6)..(6): X at position 6 is A or E
  MISC_FEATURE (11)..(11): X at position 11 is A or E
LDLLLXFIMMXL

SEQ ID NO: 148 - protein, 12 aa, Artificial
  Synthetic peptide
  MISC_FEATURE (9)..(9): X at position 9 is A or E
  MISC_FEATURE (10)..(10): X at position 10 is A or E
LDLLLMFIXXML

SEQ ID NO: 149 - protein, 12 aa, Artificial
  Synthetic peptide
  MISC_FEATURE (9)..(9): X at position 9 is A or E
  MISC_FEATURE (11)..(11): X at position 11 is A or E
LDLLLMFIXMXL

SEQ ID NO: 150 - protein, 12 aa, Artificial
  Synthetic peptide
  MISC_FEATURE (10)..(10): X at position 10 is A or E
  MISC_FEATURE (11)..(11): X at position 11 is A or E
LDLLLMFIMXXL

SEQ ID NO: 151 - protein, 12 aa, Artificial
  Synthetic peptide
  MISC_FEATURE (9)..(9): X at position 9 is A or E
  MISC_FEATURE (10)..(10): X at position 10 is A or E
  MISC_FEATURE (11)..(11): X at position 11 is A or E
LDLLLMFIXXXL

SEQ ID NO: 152 - protein, 12 aa, Artificial
  Synthetic peptide
  MISC_FEATURE (6)..(6): X at position 6 is A or E
  MISC_FEATURE (10)..(10): X at position 10 is A or E
  MISC_FEATURE (11)..(11): X at position 11 is A or E
LDLLLXFIMXXL

SEQ ID NO: 153 - protein, 12 aa, Artificial
  Synthetic peptide
  MISC_FEATURE (6)..(6): X at position 6 is A or E
  MISC_FEATURE (9)..(9): X at position 9 is A or E
  MISC_FEATURE (11)..(11): X at position 11 is A or E
LDLLLXFIXMXL

SEQ ID NO: 154 - protein, 12 aa, Artificial
  Synthetic peptide
  MISC_FEATURE (6)..(6): X at position 6 is A or E
  MISC_FEATURE (9)..(9): X at position 9 is A or E
  MISC_FEATURE (10)..(10): X at position 10 is A or E
LDLLLXFIXXML

SEQ ID NO: 155 - protein, 12 aa, Artificial
  Synthetic peptide
  MISC_FEATURE (6)..(6): X at position 6 is A or E
  MISC_FEATURE (9)..(9): X at position 9 is A or E
  MISC_FEATURE (10)..(10): X at position 10 is A or E
  MISC_FEATURE (11)..(11): X at position 11 is A or E
LDLLLXFIXXXL

SEQ ID NO: 156 - protein, 13 aa, Artificial
  Synthetic peptide
  MISC_FEATURE (7)..(7): X at position 7 is A or E
LDQLLLXFIMMML

SEQ ID NO: 157 - protein, 13 aa, Artificial
  Synthetic peptide
  MISC_FEATURE (10)..(10): X at position 10 is A or E
LDQLLLMFIXMML

SEQ ID NO: 158 - protein, 13 aa, Artificial
  Synthetic peptide
  MISC_FEATURE (11)..(11): X at position 11 is A or E
LDQLLLMFIMXML

SEQ ID NO: 159 - protein, 13 aa, Artificial
  Synthetic peptide
  MISC_FEATURE (12)..(12): X at position 12 is A or E
LDQLLLMFIMMXL

SEQ ID NO: 160 - protein, 13 aa, Artificial
  Synthetic peptide
  MISC_FEATURE (7)..(7): X at position 7 is A or E
  MISC_FEATURE (10)..(10): X at position 10 is A or E
LDQLLLXFIXMML

SEQ ID NO: 161 - protein, 13 aa, Artificial
  Synthetic peptide
  MISC_FEATURE (7)..(7): X at position 7 is A or E
  MISC_FEATURE (11)..(11): X at position 11 is A or E
LDQLLLXFIMXML

SEQ ID NO: 162 - protein, 13 aa, Artificial
  Synthetic peptide
  MISC_FEATURE (7)..(7): X at position 7 is A or E
  MISC_FEATURE (12)..(12): X at position 12 is A or E
LDQLLLXFIMMXL

SEQ ID NO: 163 - protein, 13 aa, Artificial
  Synthetic peptide
  MISC_FEATURE (10)..(10): X at position 10 is A or E
  MISC_FEATURE (11)..(11): X at position 11 is A or E
LDQLLLMFIXXML

SEQ ID NO: 164 - protein, 13 aa, Artificial
  Synthetic peptide
  MISC_FEATURE (10)..(10): X at position 10 is A or E
  MISC_FEATURE (12)..(12): X at position 12 is A or E
LDQLLLMFIXMXL

SEQ ID NO: 165 - protein, 13 aa, Artificial
  Synthetic peptide
  MISC_FEATURE (11)..(11): X at position 11 is A or E
  MISC_FEATURE (12)..(12): X at position 12 is A or E
LDQLLLMFIMXXL

SEQ ID NO: 166 - protein, 13 aa, Artificial
  Synthetic peptide
  MISC_FEATURE (10)..(10): X at position 10 is A or E
  MISC_FEATURE (11)..(11): X at position 11 is A or E
  MISC_FEATURE (12)..(12): X at position 12 is A or E
LDQLLLMFIXXXL

SEQ ID NO: 167 - protein, 13 aa, Artificial
  Synthetic peptide
  MISC_FEATURE (7)..(7): X at position 7 is A or E
  MISC_FEATURE (11)..(11): X at position 11 is A or E
  MISC_FEATURE (12)..(12): X at position 12 is A or E
LDQLLLXFIMXXL

SEQ ID NO: 168 - protein, 13 aa, Artificial
  Synthetic peptide
  MISC_FEATURE (7)..(7): X at position 7 is A or E
  MISC_FEATURE (10)..(10): X at position 10 is A or E
  MISC_FEATURE (12)..(12): X at position 12 is A or E
LDQLLLXFIXMXL

SEQ ID NO: 169 - protein, 13 aa, Artificial
  Synthetic peptide
  MISC_FEATURE (7)..(7): X at position 7 is A or E
  MISC_FEATURE (10)..(10): X at position 10 is A or E
  MISC_FEATURE (11)..(11): X at position 11 is A or E
LDQLLLXFIXXML

SEQ ID NO: 170 - protein, 13 aa, Artificial
  Synthetic peptide
  MISC_FEATURE (7)..(7): X at position 7 is A or E
  MISC_FEATURE (10)..(10): X at position 10 is A or E
  MISC_FEATURE (11)..(11): X at position 11 is A or E
  MISC_FEATURE (12)..(12): X at position 12 is A or E
LDQLLLXFIXXXL

SEQ ID NO: 171 - protein, 12 aa, Artificial
  Synthetic peptide
  MISC_FEATURE (1)..(1): X at position 1 is E or V
XDLLLMFIMMML

SEQ ID NO: 172 - protein, 12 aa, Artificial
  Synthetic peptide
  MISC_FEATURE (1)..(1): X at position 1 is E or V
  MISC_FEATURE (6)..(6): X at position 6 is A or E
XDLLLXFIMMML

SEQ ID NO: 173 - protein, 12 aa, Artificial
  Synthetic peptide
  MISC_FEATURE (1)..(1): X at position 1 is E or V
  MISC_FEATURE (9)..(9): X at position 9 is A or E
XDLLLMFIXMML

SEQ ID NO: 174 - protein, 12 aa, Artificial
  Synthetic peptide
  MISC_FEATURE (1)..(1): X at position 1 is E or V
  MISC_FEATURE (10)..(10): X at position 10 is A or E
XDLLLMFIMXML

SEQ ID NO: 175 - protein, 12 aa, Artificial
  Synthetic peptide
  MISC_FEATURE (1)..(1): X at position 1 is E or V
  MISC_FEATURE (11)..(11): X at position 11 is A or E
XDLLLMFIMMXL

SEQ ID NO: 176 - protein, 12 aa, Artificial
  Synthetic peptide
  MISC_FEATURE (1)..(1): X at position 1 is E or V
  MISC_FEATURE (6)..(6): X at position 6 is A or E
  MISC_FEATURE (9)..(9): X at position 9 is A or E
XDLLLXFIXMML

SEQ ID NO: 177 - protein, 12 aa, Artificial
  Synthetic peptide
  MISC_FEATURE (1)..(1): X at position 1 is E or V
  MISC_FEATURE (6)..(6): X at position 6 is A or E
  MISC_FEATURE (10)..(10): X at position 10 is A or E
XDLLLXFIMXML

SEQ ID NO: 178 - protein, 12 aa, Artificial
  Synthetic peptide
  MISC_FEATURE (1)..(1): X at position 1 is E or V
  MISC_FEATURE (6)..(6): X at position 6 is A or E
  MISC_FEATURE (11)..(11): X at position 11 is A or E
XDLLLXFIMMXL

SEQ ID NO: 179 - protein, 12 aa, Artificial
  Synthetic peptide
  MISC_FEATURE (1)..(1): X at position 1 is E or V
  MISC_FEATURE (9)..(9): X at position 9 is A or E
  MISC_FEATURE (10)..(10): X at position 10 is A or E
XDLLLMFIXXML

SEQ ID NO: 180 - protein, 12 aa, Artificial
  Synthetic peptide
  MISC_FEATURE (1)..(1): X at position 1 is E or V
  MISC_FEATURE (9)..(9): X at position 9 is A or E
  MISC_FEATURE (11)..(11): X at position 11 is A or E
XDLLLMFIXMXL

SEQ ID NO: 181 - protein, 12 aa, Artificial
  Synthetic peptide
  MISC_FEATURE (1)..(1): X at position 1 is E or V
  MISC_FEATURE (10)..(10): X at position 10 is A or E
  MISC_FEATURE (11)..(11): X at position 11 is A or E
XDLLLMFIMXXL

SEQ ID NO: 182 - protein, 12 aa, Artificial
  Synthetic peptide
  MISC_FEATURE (1)..(1): X at position 1 is E or V
  MISC_FEATURE (9)..(9): X at position 9 is A or E
  MISC_FEATURE (10)..(10): X at position 10 is A or E
  MISC_FEATURE (11)..(11): X at position 11 is A or E
XDLLLMFIXXXL

SEQ ID NO: 183 - protein, 12 aa, Artificial
  Synthetic peptide
  MISC_FEATURE (1)..(1): X at position 1 is E or V
  MISC_FEATURE (6)..(6): X at position 6 is A or E
  MISC_FEATURE (10)..(10): X at position 10 is A or E
  MISC_FEATURE (11)..(11): X at position 11 is A or E
XDLLLXFIMXXL

SEQ ID NO: 184 - protein, 12 aa, Artificial
  Synthetic peptide
  MISC_FEATURE (1)..(1): X at position 1 is E or V
  MISC_FEATURE (6)..(6): X at position 6 is A or E
  MISC_FEATURE (9)..(9): X at position 9 is A or E
  MISC_FEATURE (11)..(11): X at position 11 is A or E
XDLLLXFIXMXL

SEQ ID NO: 185 - protein, 12 aa, Artificial
  Synthetic peptide
  MISC_FEATURE (1)..(1): X at position 1 is E or V
  MISC_FEATURE (6)..(6): X at position 6 is A or E
  MISC_FEATURE (9)..(9): X at position 9 is A or E
  MISC_FEATURE (10)..(10): X at position 10 is A or E
XDLLLXFIXXML

SEQ ID NO: 186 - protein, 12 aa, Artificial
  Synthetic peptide
  MISC_FEATURE (1)..(1): X at position 1 is E or V
  MISC_FEATURE (6)..(6): X at position 6 is A or E
  MISC_FEATURE (9)..(9): X at position 9 is A or E
  MISC_FEATURE (10)..(10): X at position 10 is A or E
  MISC_FEATURE (11)..(11): X at position 11 is A or E
XDLLLXFIXXXL

SEQ ID NO: 187 - protein, 13 aa, Artificial
  Synthetic peptide
  MISC_FEATURE (1)..(1): X at position 1 is E or V
XDQLLLMFIMMML

SEQ ID NO: 188 - protein, 13 aa, Artificial
  Synthetic peptide
  MISC_FEATURE (1)..(1): X at position 1 is E or V
  MISC_FEATURE (7)..(7): X at position 7 is A or E
XDQLLLXFIMMML

SEQ ID NO: 189 - protein, 13 aa, Artificial
  Synthetic peptide
  MISC_FEATURE (1)..(1): X at position 1 is E or V
  MISC_FEATURE (10)..(10): X at position 10 is A or E
XDQLLLMFIXMML

SEQ ID NO: 190 - protein, 13 aa, Artificial
  Synthetic peptide
  MISC_FEATURE (1)..(1): X at position 1 is E or V
  MISC_FEATURE (11)..(11): X at position 11 is A or E
XDQLLLMFIMXML

SEQ ID NO: 191 - protein, 13 aa, Artificial
  Synthetic peptide
  MISC_FEATURE (1)..(1): X at position 1 is E or V
  MISC_FEATURE (12)..(12): X at position 12 is A or E
XDQLLLMFIMMXL

SEQ ID NO: 192 - protein, 13 aa, Artificial
  Synthetic peptide
  MISC_FEATURE (1)..(1): X at position 1 is E or V
  MISC_FEATURE (7)..(7): X at position 7 is A or E
  MISC_FEATURE (10)..(10): X at position 10 is A or E
XDQLLLXFIXMML

SEQ ID NO: 193 - protein, 13 aa, Artificial
  Synthetic peptide
  MISC_FEATURE (1)..(1): X at position 1 is E or V
  MISC_FEATURE (7)..(7): X at position 7 is A or E
  MISC_FEATURE (11)..(11): X at position 11 is A or E
XDQLLLXFIMXML

SEQ ID NO: 194 - protein, 13 aa, Artificial
  Synthetic peptide
  MISC_FEATURE (1)..(1): X at position 1 is E or V
  MISC_FEATURE (7)..(7): X at position 7 is A or E
  MISC_FEATURE (12)..(12): X at position 12 is A or E
XDQLLLXFIMMXL

SEQ ID NO: 195 - protein, 13 aa, Artificial
  Synthetic peptide
  MISC_FEATURE (1)..(1): X at position 1 is E or V
  MISC_FEATURE (10)..(10): X at position 10 is A or E
  MISC_FEATURE (11)..(11): X at position 11 is A or E
XDQLLLMFIXXML

SEQ ID NO: 196 - protein, 13 aa, Artificial
  Synthetic peptide
  MISC_FEATURE (1)..(1): X at position 1 is E or V
  MISC_FEATURE (10)..(10): X at position 10 is A or E
  MISC_FEATURE (12)..(12): X at position 12 is A or E
XDQLLLMFIXMXL

SEQ ID NO: 197 - protein, 13 aa, Artificial
  Synthetic peptide
  MISC_FEATURE (1)..(1): X at position 1 is E or V
  MISC_FEATURE (11)..(11): X at position 11 is A or E
  MISC_FEATURE (12)..(12): X at position 12 is A or E
XDQLLLMFIMXXL

SEQ ID NO: 198 - protein, 13 aa, Artificial
  Synthetic peptide
  MISC_FEATURE (1)..(1): X at position 1 is E or V
  MISC_FEATURE (10)..(10): X at position 10 is A or E
  MISC_FEATURE (11)..(11): X at position 11 is A or E
  MISC_FEATURE (12)..(12): X at position 12 is A or E
XDQLLLMFIXXXL

SEQ ID NO: 199 - protein, 13 aa, Artificial
  Synthetic peptide
  MISC_FEATURE (1)..(1): X at position 1 is E or V
  MISC_FEATURE (7)..(7): X at position 7 is A or E
  MISC_FEATURE (11)..(11): X at position 11 is A or E
  MISC_FEATURE (12)..(12): X at position 12 is A or E
XDQLLLXFIMXXL

SEQ ID NO: 200 - protein, 13 aa, Artificial
  Synthetic peptide
  MISC_FEATURE (1)..(1): X at position 1 is E or V
  MISC_FEATURE (7)..(7): X at position 7 is A or E
  MISC_FEATURE (10)..(10): X at position 10 is A or E
  MISC_FEATURE (12)..(12): X at position 12 is A or E
XDQLLLXFIXMXL

SEQ ID NO: 201 - protein, 13 aa, Artificial
  Synthetic peptide
  MISC_FEATURE (1)..(1): X at position 1 is E or V
  MISC_FEATURE (7)..(7): X at position 7 is A or E
  MISC_FEATURE (10)..(10): X at position 10 is A or E
  MISC_FEATURE (11)..(11): X at position 11 is A or E
XDQLLLXFIXXML

SEQ ID NO: 202 - protein, 13 aa, Artificial
  Synthetic peptide
  MISC_FEATURE (1)..(1): X at position 1 is E or V
  MISC_FEATURE (7)..(7): X at position 7 is A or E
  MISC_FEATURE (10)..(10): X at position 10 is A or E
  MISC_FEATURE (11)..(11): X at position 11 is A or E
  MISC_FEATURE (12)..(12): X at position 12 is A or E
XDQLLLXFIXXXL

SEQ ID NO: 203 - protein, 12 aa, Artificial
  Synthetic peptide
  MISC_FEATURE (3)..(3): X at position 3 is E or V
LDXLLMFIMMML

SEQ ID NO: 204 - protein, 12 aa, Artificial
  Synthetic peptide
  MISC_FEATURE (3)..(3): X at position 3 is E or V
  MISC_FEATURE (6)..(6): X at position 6 is A or E
LDXLLXFIMMML

SEQ ID NO: 205 - protein, 12 aa, Artificial
  Synthetic peptide
  MISC_FEATURE (3)..(3): X at position 3 is E or V
  MISC_FEATURE (9)..(9): X at position 9 is A or E
LDXLLMFIXMML

SEQ ID NO: 206 - protein, 12 aa, Artificial
  Synthetic peptide
  MISC_FEATURE (3)..(3): X at position 3 is E or V
  MISC_FEATURE (10)..(10): X at position 10 is A or E
LDXLLMFIMXML

SEQ ID NO: 207 - protein, 12 aa, Artificial
  Synthetic peptide
  MISC_FEATURE (3)..(3): X at position 3 is E or V
  MISC_FEATURE (11)..(11): X at position 11 is A or E
LDXLLMFIMMXL

SEQ ID NO: 208 - protein, 12 aa, Artificial
  Synthetic peptide
  MISC_FEATURE (3)..(3): X at position 3 is E or V
  MISC_FEATURE (6)..(6): X at position 6 is A or E
  MISC_FEATURE (9)..(9): X at position 9 is A or E
LDXLLXFIXMML

SEQ ID NO: 209 - protein, 12 aa, Artificial
  Synthetic peptide
  MISC_FEATURE (3)..(3): X at position 3 is E or V
  MISC_FEATURE (6)..(6): X at position 6 is A or E
  MISC_FEATURE (10)..(10): X at position 10 is A or E
LDXLLXFIMXML

SEQ ID NO: 210 - protein, 12 aa, Artificial
  Synthetic peptide
  MISC_FEATURE (3)..(3): X at position 3 is E or V
  MISC_FEATURE (6)..(6): X at position 6 is A or E
  MISC_FEATURE (11)..(11): X at position 11 is A or E
LDXLLXFIMMXL

SEQ ID NO: 211 - protein, 12 aa, Artificial
  Synthetic peptide
  MISC_FEATURE (3)..(3): X at position 3 is E or V
  MISC_FEATURE (9)..(9): X at position 9 is A or E
  MISC_FEATURE (10)..(10): X at position 10 is A or E
LDXLLMFIXXML

SEQ ID NO: 212 - protein, 12 aa, Artificial
  Synthetic peptide
  MISC_FEATURE (3)..(3): X at position 3 is E or V
  MISC_FEATURE (9)..(9): X at position 9 is A or E
  MISC_FEATURE (11)..(11): X at position 11 is A or E
LDXLLMFIXMXL

SEQ ID NO: 213 - protein, 12 aa, Artificial
  Synthetic peptide
  MISC_FEATURE (3)..(3): X at position 3 is E or V
  MISC_FEATURE (10)..(10): X at position 10 is A or E
  MISC_FEATURE (11)..(11): X at position 11 is A or E
LDXLLMFIMXXL

SEQ ID NO: 214 - protein, 12 aa, Artificial
  Synthetic peptide
  MISC_FEATURE (3)..(3): X at position 3 is E or V
  MISC_FEATURE (9)..(9): X at position 9 is A or E
  MISC_FEATURE (10)..(10): X at position 10 is A or E
  MISC_FEATURE (11)..(11): X at position 11 is A or E
LDXLLMFIXXXL

SEQ ID NO: 215 - protein, 12 aa, Artificial
  Synthetic peptide
  MISC_FEATURE (3)..(3): X at position 3 is E or V
  MISC_FEATURE (6)..(6): X at position 6 is A or E
  MISC_FEATURE (10)..(10): X at position 10 is A or E
  MISC_FEATURE (11)..(11): X at position 11 is A or E
LDXLLXFIMXXL

SEQ ID NO: 216 - protein, 12 aa, Artificial
  Synthetic peptide
  MISC_FEATURE (3)..(3): X at position 3 is E or V
  MISC_FEATURE (6)..(6): X at position 6 is A or E
  MISC_FEATURE (9)..(9): X at position 9 is A or E
  MISC_FEATURE (11)..(11): X at position 11 is A or E
LDXLLXFIXMXL

SEQ ID NO: 217 - protein, 12 aa, Artificial
  Synthetic peptide
  MISC_FEATURE (3)..(3): X at position 3 is E or V
  MISC_FEATURE (6)..(6): X at position 6 is A or E
  MISC_FEATURE (9)..(9): X at position 9 is A or E
  MISC_FEATURE (10)..(10): X at position 10 is A or E
LDXLLXFIXXML

SEQ ID NO: 218 - protein, 12 aa, Artificial
  Synthetic peptide
  MISC_FEATURE (3)..(3): X at position 3 is E or V
  MISC_FEATURE (6)..(6): X at position 6 is A or E
  MISC_FEATURE (9)..(9): X at position 9 is A or E
  MISC_FEATURE (10)..(10): X at position 10 is A or E
  MISC_FEATURE (11)..(11): X at position 11 is A or E
LDXLLXFIXXXL

SEQ ID NO: 219 - protein, 13 aa, Artificial
  Synthetic peptide
  MISC_FEATURE (4)..(4): X at position 4 is E or V
LDQXLLMFIMMML

SEQ ID NO: 220 - protein, 13 aa, Artificial
  Synthetic peptide
  MISC_FEATURE (4)..(4): X at position 4 is E or V
  MISC_FEATURE (7)..(7): X at position 7 is A or E
LDQXLLXFIMMML

SEQ ID NO: 221 - protein, 13 aa, Artificial
  Synthetic peptide
  MISC_FEATURE (4)..(4): X at position 4 is E or V
  MISC_FEATURE (10)..(10): X at position 10 is A or E
LDQXLLMFIXMML

SEQ ID NO: 222 - protein, 13 aa, Artificial
  Synthetic peptide
  MISC_FEATURE (4)..(4): X at position 4 is E or V
  MISC_FEATURE (11)..(11): X at position 11 is A or E
LDQXLLMFIMXML

SEQ ID NO: 223 - protein, 13 aa, Artificial
  Synthetic peptide
  MISC_FEATURE (4)..(4): X at position 4 is E or V
  MISC_FEATURE (12)..(12): X at position 12 is A or E
LDQXLLMFIMMXL

SEQ ID NO: 224 - protein, 13 aa, Artificial
  Synthetic peptide
  MISC_FEATURE (4)..(4): X at position 4 is E or V
  MISC_FEATURE (7)..(7): X at position 7 is A or E
  MISC_FEATURE (10)..(10): X at position 10 is A or E
LDQXLLXFIXMML

SEQ ID NO: 225 - protein, 13 aa, Artificial
  Synthetic peptide
  MISC_FEATURE (4)..(4): X at position 4 is E or V
  MISC_FEATURE (7)..(7): X at position 7 is A or E
  MISC_FEATURE (11)..(11): X at position 11 is A or E
LDQXLLXFIMXML

SEQ ID NO: 226 - protein, 13 aa, Artificial
  Synthetic peptide
  MISC_FEATURE (4)..(4): X at position 4 is E or V
  MISC_FEATURE (7)..(7): X at position 7 is A or E
  MISC_FEATURE (12)..(12): X at position 12 is A or E
LDQXLLXFIMMXL

SEQ ID NO: 227 - protein, 13 aa, Artificial
  Synthetic peptide
  MISC_FEATURE (4)..(4): X at position 4 is E or V
  MISC_FEATURE (10)..(10): X at position 10 is A or E
  MISC_FEATURE (11)..(11): X at position 11 is A or E
LDQXLLMFIXXML

SEQ ID NO: 228 - protein, 13 aa, Artificial
  Synthetic peptide
  MISC_FEATURE (4)..(4): X at position 4 is E or V
  MISC_FEATURE (10)..(10): X at position 10 is A or E
  MISC_FEATURE (12)..(12): X at position 12 is A or E
LDQXLLMFIXMXL

SEQ ID NO: 229 - protein, 13 aa, Artificial
  Synthetic peptide
  MISC_FEATURE (4)..(4): X at position 4 is E or V
  MISC_FEATURE (11)..(11): X at position 11 is A or E
  MISC_FEATURE (12)..(12): X at position 12 is A or E
LDQXLLMFIMXXL

SEQ ID NO: 230 - protein, 13 aa, Artificial
  Synthetic peptide
  MISC_FEATURE (4)..(4): X at position 4 is E or V
  MISC_FEATURE (10)..(10): X at position 10 is A or E
  MISC_FEATURE (11)..(11): X at position 11 is A or E
  MISC_FEATURE (12)..(12): X at position 12 is A or E
LDQXLLMFIXXXL

SEQ ID NO: 231 - protein, 13 aa, Artificial
  Synthetic peptide
  MISC_FEATURE (4)..(4): X at position 4 is E or V
  MISC_FEATURE (7)..(7): X at position 7 is A or E
  MISC_FEATURE (11)..(11): X at position 11 is A or E
  MISC_FEATURE (12)..(12): X at position 12 is A or E
LDQXLLXFIMXXL

SEQ ID NO: 232 - protein, 13 aa, Artificial
  Synthetic peptide
  MISC_FEATURE (4)..(4): X at position 4 is E or V
  MISC_FEATURE (7)..(7): X at position 7 is A or E
  MISC_FEATURE (10)..(10): X at position 10 is A or E
  MISC_FEATURE (12)..(12): X at position 12 is A or E
LDQXLLXFIXMXL

SEQ ID NO: 233 - protein, 13 aa, Artificial
  Synthetic peptide
  MISC_FEATURE (4)..(4): X at position 4 is E or V
  MISC_FEATURE (7)..(7): X at position 7 is A or E
  MISC_FEATURE (10)..(10): X at position 10 is A or E
  MISC_FEATURE (11)..(11): X at position 11 is A or E
LDQXLLXFIXXML

SEQ ID NO: 234 - protein, 13 aa, Artificial
  Synthetic peptide
  MISC_FEATURE (4)..(4): X at position 4 is E or V
  MISC_FEATURE (7)..(7): X at position 7 is A or E
  MISC_FEATURE (10)..(10): X at position 10 is A or E
  MISC_FEATURE (11)..(11): X at position 11 is A or E
  MISC_FEATURE (12)..(12): X at position 12 is A or E
LDQXLLXFIXXXL

SEQ ID NO: 235 - protein, 12 aa, Artificial
  Synthetic peptide
  MISC_FEATURE (4)..(4): X at position 4 is E or V
LDLXLMFIMMML

SEQ ID NO: 236 - protein, 12 aa, Artificial
  Synthetic peptide
  MISC_FEATURE (4)..(4): X at position 4 is E or V
  MISC_FEATURE (6)..(6): X at position 6 is A or E
LDLXLXFIMMML

SEQ ID NO: 237 - protein, 12 aa, Artificial
  Synthetic peptide
  MISC_FEATURE (4)..(4): X at position 4 is E or V
  MISC_FEATURE (9)..(9): X at position 9 is A or E
LDLXLMFIXMML

SEQ ID NO: 238 - protein, 12 aa, Artificial
  Synthetic peptide
  MISC_FEATURE (4)..(4): X at position 4 is E or V
  MISC_FEATURE (10)..(10): X at position 10 is A or E
LDLXLMFIMXML

SEQ ID NO: 239 - protein, 12 aa, Artificial
  Synthetic peptide
  MISC_FEATURE (4)..(4): X at position 4 is E or V
  MISC_FEATURE (11)..(11): X at position 11 is A or E
LDLXLMFIMMXL

SEQ ID NO: 240 - protein, 12 aa, Artificial
  Synthetic peptide
  MISC_FEATURE (4)..(4): X at position 4 is E or V
  MISC_FEATURE (6)..(6): X at position 6 is A or E
  MISC_FEATURE (9)..(9): X at position 9 is A or E
LDLXLXFIXMML

SEQ ID NO: 241 - protein, 12 aa, Artificial
  Synthetic peptide
  MISC_FEATURE (4)..(4): X at position 4 is E or V
  MISC_FEATURE (6)..(6): X at position 6 is A or E
  MISC_FEATURE (10)..(10): X at position 10 is A or E
LDLXLXFIMXML

SEQ ID NO: 242 - protein, 12 aa, Artificial
  Synthetic peptide
  MISC_FEATURE (4)..(4): X at position 4 is E or V
  MISC_FEATURE (6)..(6): X at position 6 is A or E
  MISC_FEATURE (11)..(11): X at position 11 is A or E
LDLXLXFIMMXL

SEQ ID NO: 243 - protein, 12 aa, Artificial
  Synthetic peptide
  MISC_FEATURE (4)..(4): X at position 4 is E or V
  MISC_FEATURE (9)..(9): X at position 9 is A or E
  MISC_FEATURE (10)..(10): X at position 10 is A or E
LDLXLMFIXXML

SEQ ID NO: 244 - protein, 12 aa, Artificial
  Synthetic peptide
  MISC_FEATURE (4)..(4): X at position 4 is E or V
  MISC_FEATURE (9)..(9): X at position 9 is A or E
  MISC_FEATURE (11)..(11): X at position 11 is A or E
LDLXLMFIXMXL

SEQ ID NO: 245 - protein, 12 aa, Artificial
  Synthetic peptide
  MISC_FEATURE (4)..(4): X at position 4 is E or V
  MISC_FEATURE (10)..(10): X at position 10 is A or E
  MISC_FEATURE (11)..(11): X at position 11 is A or E
LDLXLMFIMXXL

SEQ ID NO: 246 - protein, 12 aa, Artificial
  Synthetic peptide
  MISC_FEATURE (4)..(4): X at position 4 is E or V
  MISC_FEATURE (9)..(9): X at position 9 is A or E
  MISC_FEATURE (10)..(10): X at position 10 is A or E
  MISC_FEATURE (11)..(11): X at position 11 is A or E
LDLXLMFIXXXL

SEQ ID NO: 247 - protein, 13 aa, Artificial
  Synthetic peptide
  MISC_FEATURE (4)..(4): X at position 4 is E or V
  MISC_FEATURE (7)..(7): X at position 7 is A or E
  MISC_FEATURE (11)..(11): X at position 11 is A or E
  MISC_FEATURE (12)..(12): X at position 12 is A or E
LDLXLLXFIMXXL

SEQ ID NO: 248 - protein, 13 aa, Artificial
  Synthetic peptide
  MISC_FEATURE (4)..(4): X at position 4 is E or V
  MISC_FEATURE (7)..(7): X at position 7 is A or E
  MISC_FEATURE (10)..(10): X at position 10 is A or E
  MISC_FEATURE (12)..(12): X at position 12 is A or E
LDLXLLXFIXMXL

SEQ ID NO: 249 - protein, 13 aa, Artificial
  Synthetic peptide
  MISC_FEATURE (4)..(4): X at position 4 is E or V
  MISC_FEATURE (7)..(7): X at position 7 is A or E
  MISC_FEATURE (10)..(10): X at position 10 is A or E
  MISC_FEATURE (11)..(11): X at position 11 is A or E
LDLXLLXFIXXML

SEQ ID NO: 250 - protein, 12 aa, Artificial
  Synthetic peptide
  MISC_FEATURE (4)..(4): X at position 4 is E or V
  MISC_FEATURE (6)..(6): X at position 6 is A or E
  MISC_FEATURE (9)..(9): X at position 9 is A or E
  MISC_FEATURE (10)..(10): X at position 10 is A or E
  MISC_FEATURE (11)..(11): X at position 11 is A or E
LDLXLXFIXXXL

SEQ ID NO: 251 - protein, 13 aa, Artificial
  Synthetic peptide
  MISC_FEATURE (5)..(5): X at position 5 is E or V
LDQLXLMFIMMML

SEQ ID NO: 252 - protein, 13 aa, Artificial
  Synthetic peptide
  MISC_FEATURE (5)..(5): X at position 5 is E or V
  MISC_FEATURE (7)..(7): X at position 7 is A or E
LDQLXLXFIMMML

SEQ ID NO: 253 - protein, 13 aa, Artificial
  Synthetic peptide
  MISC_FEATURE (5)..(5): X at position 5 is E or V
  MISC_FEATURE (10)..(10): X at position 10 is A or E
LDQLXLMFIXMML

SEQ ID NO: 254 - protein, 13 aa, Artificial
  Synthetic peptide
  MISC_FEATURE (5)..(5): X at position 5 is E or V
  MISC_FEATURE (11)..(11): X at position 11 is A or E
LDQLXLMFIMXML

SEQ ID NO: 255 - protein, 13 aa, Artificial
  Synthetic peptide
  MISC_FEATURE (5)..(5): X at position 5 is E or V
  MISC_FEATURE (12)..(12): X at position 12 is A or E
LDQLXLMFIMMXL

SEQ ID NO: 256 - protein, 13 aa, Artificial
  Synthetic peptide
  MISC_FEATURE (5)..(5): X at position 5 is E or V
  MISC_FEATURE (7)..(7): X at position 7 is A or E
  MISC_FEATURE (10)..(10): X at position 10 is A or E
LDQLXLXFIXMML

SEQ ID NO: 257 - protein, 13 aa, Artificial
  Synthetic peptide
  MISC_FEATURE (5)..(5): X at position 5 is E or V
  MISC_FEATURE (7)..(7): X at position 7 is A or E
  MISC_FEATURE (11)..(11): X at position 11 is A or E
LDQLXLXFIMXML

SEQ ID NO: 258 - protein, 13 aa, Artificial
  Synthetic peptide
  MISC_FEATURE (5)..(5): X at position 5 is E or V
  MISC_FEATURE (7)..(7): X at position 7 is A or E
  MISC_FEATURE (12)..(12): X at position 12 is A or E
LDQLXLXFIMMXL

SEQ ID NO: 259 - protein, 13 aa, Artificial
  Synthetic peptide
  MISC_FEATURE (5)..(5): X at position 5 is E or V
  MISC_FEATURE (10)..(10): X at position 10 is A or E
  MISC_FEATURE (11)..(11): X at position 11 is A or E
LDQLXLMFIXXML

SEQ ID NO: 260 - protein, 13 aa, Artificial
  Synthetic peptide
  MISC_FEATURE (5)..(5): X at position 5 is E or V
  MISC_FEATURE (10)..(10): X at position 10 is A or E
  MISC_FEATURE (12)..(12): X at position 12 is A or E
LDQLXLMFIXMXL

SEQ ID NO: 261 - protein, 13 aa, Artificial
  Synthetic peptide
  MISC_FEATURE (5)..(5): X at position 5 is E or V
  MISC_FEATURE (11)..(11): X at position 11 is A or E
  MISC_FEATURE (12)..(12): X at position 12 is A or E
LDQLXLMFIMXXL

SEQ ID NO: 262 - protein, 13 aa, Artificial
  Synthetic peptide
  MISC_FEATURE (5)..(5): X at position 5 is E or V
  MISC_FEATURE (10)..(10): X at position 10 is A or E
  MISC_FEATURE (11)..(11): X at position 11 is A or E
  MISC_FEATURE (12)..(12): X at position 12 is A or E
LDQLXLMFIXXXL

SEQ ID NO: 263 - protein, 14 aa, Artificial
  Synthetic peptide
  MISC_FEATURE (5)..(5): X at position 5 is E or V
  MISC_FEATURE (8)..(8): X at position 8 is A or E
  MISC_FEATURE (12)..(12): X at position 12 is A or E
  MISC_FEATURE (13)..(13): X at position 13 is A or E
LDQLXLLXFIMXXL

SEQ ID NO: 264 - protein, 14 aa, Artificial
  Synthetic peptide
  MISC_FEATURE (5)..(5): X at position 5 is E or V
  MISC_FEATURE (8)..(8): X at position 8 is A or E
  MISC_FEATURE (11)..(11): X at position 11 is A or E
  MISC_FEATURE (13)..(13): X at position 13 is A or E
LDQLXLLXFIXMXL

SEQ ID NO: 265 - protein, 14 aa, Artificial
  Synthetic peptide
  MISC_FEATURE (5)..(5): X at position 5 is E or V
  MISC_FEATURE (8)..(8): X at position 8 is A or E
  MISC_FEATURE (11)..(11): X at position 11 is A or E
  MISC_FEATURE (12)..(12): X at position 12 is A or E
LDQLXLLXFIXXML

SEQ ID NO: 266 - protein, 13 aa, Artificial
  Synthetic peptide
  MISC_FEATURE (5)..(5): X at position 5 is E or V
  MISC_FEATURE (7)..(7): X at position 7 is A or E
  MISC_FEATURE (10)..(10): X at position 10 is A or E
  MISC_FEATURE (11)..(11): X at position 11 is A or E
  MISC_FEATURE (12)..(12): X at position 12 is A or E
LDQLXLXFIXXXL

SEQ ID NO: 267 - protein, 12 aa, Artificial
  Synthetic peptide
  MISC_FEATURE (5)..(5): X at position 5 is E or V
LDLLXMFIMMML

SEQ ID NO: 268 - protein, 12 aa, Artificial
  Synthetic peptide
  MISC_FEATURE (5)..(5): X at position 5 is E or V
  MISC_FEATURE (6)..(6): X at position 6 is A or E
LDLLXXFIMMML

SEQ ID NO: 269 - protein, 12 aa, Artificial
  Synthetic peptide
  MISC_FEATURE (5)..(5): X at position 5 is E or V
  MISC_FEATURE (9)..(9): X at position 9 is A or E
LDLLXMFIXMML

SEQ ID NO: 270 - protein, 12 aa, Artificial
  Synthetic peptide
  MISC_FEATURE (5)..(5): X at position 5 is E or V
  MISC_FEATURE (10)..(10): X at position 10 is A or E
LDLLXMFIMXML

SEQ ID NO: 271 - protein, 12 aa, Artificial
  Synthetic peptide
  MISC_FEATURE (5)..(5): X at position 5 is E or V
  MISC_FEATURE (11)..(11): X at position 11 is A or E
LDLLXMFIMMXL

SEQ ID NO: 272 - protein, 12 aa, Artificial
  Synthetic peptide
  MISC_FEATURE (5)..(5): X at position 5 is E or V
  MISC_FEATURE (6)..(6): X at position 6 is A or E
  MISC_FEATURE (9)..(9): X at position 9 is A or E
LDLLXXFIXMML

SEQ ID NO: 273 - protein, 12 aa, Artificial
  Synthetic peptide
  MISC_FEATURE (5)..(5): X at position 5 is E or V
  MISC_FEATURE (6)..(6): X at position 6 is A or E
  MISC_FEATURE (10)..(10): X at position 10 is A or E
LDLLXXFIMXML

SEQ ID NO: 274 - protein, 12 aa, Artificial
  Synthetic peptide
  MISC_FEATURE (5)..(5): X at position 5 is E or V
  MISC_FEATURE (6)..(6): X at position 6 is A or E
  MISC_FEATURE (11)..(11): X at position 11 is A or E
LDLLXXFIMMXL

SEQ ID NO: 275 - protein, 12 aa, Artificial
  Synthetic peptide
  MISC_FEATURE (5)..(5): X at position 5 is E or V
  MISC_FEATURE (9)..(9): X at position 9 is A or E
  MISC_FEATURE (10)..(10): X at position 10 is A or E
LDLLXMFIXXML

SEQ ID NO: 276 - protein, 12 aa, Artificial
  Synthetic peptide
  MISC_FEATURE (5)..(5): X at position 5 is E or V
  MISC_FEATURE (9)..(9): X at position 9 is A or E
  MISC_FEATURE (11)..(11): X at position 11 is A or E
LDLLXMFIXMXL

SEQ ID NO: 277 - protein, 12 aa, Artificial
  Synthetic peptide
  MISC_FEATURE (5)..(5): X at position 5 is E or V
  MISC_FEATURE (10)..(10): X at position 10 is A or E
  MISC_FEATURE (11)..(11): X at position 11 is A or E
LDLLXMFIMXXL

SEQ ID NO: 278 - protein, 12 aa, Artificial
  Synthetic peptide
  MISC_FEATURE (5)..(5): X at position 5 is E or V
  MISC_FEATURE (9)..(9): X at position 9 is A or E
  MISC_FEATURE (10)..(10): X at position 10 is A or E
  MISC_FEATURE (11)..(11): X at position 11 is A or E
LDLLXMFIXXXL

SEQ ID NO: 279 - protein, 14 aa, Artificial
  Synthetic peptide
  MISC_FEATURE (5)..(5): X at position 5 is E or V
  MISC_FEATURE (8)..(8): X at position 8 is A or E
  MISC_FEATURE (12)..(12): X at position 12 is A or E
  MISC_FEATURE (13)..(13): X at position 13 is A or E
LDLLXLLXFIMXXL

SEQ ID NO: 280 - protein, 14 aa, Artificial
  Synthetic peptide
  MISC_FEATURE (5)..(5): X at position 5 is E or V
  MISC_FEATURE (8)..(8): X at position 8 is A or E
  MISC_FEATURE (11)..(11): X at position 11 is A or E
  MISC_FEATURE (13)..(13): X at position 13 is A or E
LDLLXLLXFIXMXL

SEQ ID NO: 281 - protein, 14 aa, Artificial
  Synthetic peptide
  MISC_FEATURE (5)..(5): X at position 5 is E or V
  MISC_FEATURE (8)..(8): X at position 8 is A or E
  MISC_FEATURE (11)..(11): X at position 11 is A or E
  MISC_FEATURE (12)..(12): X at position 12 is A or E
LDLLXLLXFIXXML

SEQ ID NO: 282 - protein, 12 aa, Artificial
  Synthetic peptide
  MISC_FEATURE (5)..(5): X at position 5 is E or V
  MISC_FEATURE (6)..(6): X at position 6 is A or E
  MISC_FEATURE (9)..(9): X at position 9 is A or E
  MISC_FEATURE (10)..(10): X at position 10 is A or E
  MISC_FEATURE (11)..(11): X at position 10 is A or E
LDLLXXFIXXXL

SEQ ID NO: 283 - protein, 13 aa, Artificial
  Synthetic peptide
  MISC_FEATURE (6)..(6): X at position 6 is E or V
LDQLLXMFIMMML

SEQ ID NO: 284 - protein, 13 aa, Artificial
  Synthetic peptide
  MISC_FEATURE (6)..(6): X at position 6 is E or V
  MISC_FEATURE (7)..(7): X at position 7 is A or E
LDQLLXXFIMMML

SEQ ID NO: 285 - protein, 13 aa, Artificial
  Synthetic peptide
  MISC_FEATURE (6)..(6): X at position 6 is E or V
  MISC_FEATURE (10)..(10): X at position 10 is A or E
LDQLLXMFIXMML

SEQ ID NO: 286 - protein, 13 aa, Artificial
  Synthetic peptide
  MISC_FEATURE (6)..(6): X at position 6 is E or V
  MISC_FEATURE (11)..(11): X at position 11 is A or E
LDQLLXMFIMXML

SEQ ID NO: 287 - protein, 13 aa, Artificial
  Synthetic peptide
  MISC_FEATURE (6)..(6): X at position 6 is E or V
  MISC_FEATURE (12)..(12): X at position 12 is A or E
LDQLLXMFIMMXL

SEQ ID NO: 288 - protein, 13 aa, Artificial
  Synthetic peptide
  MISC_FEATURE (6)..(6): X at position 6 is E or V
  MISC_FEATURE (7)..(7): X at position 7 is A or E
  MISC_FEATURE (10)..(10): X at position 10 is A or E
LDQLLXXFIXMML

SEQ ID NO: 289 - protein, 13 aa, Artificial
  Synthetic peptide
  MISC_FEATURE (6)..(6): X at position 6 is E or V
  MISC_FEATURE (7)..(7): X at position 7 is A or E
  MISC_FEATURE (11)..(11): X at position 11 is A or E
LDQLLXXFIMXML

SEQ ID NO: 290 - protein, 13 aa, Artificial
  Synthetic peptide
  MISC_FEATURE (6)..(6): X at position 6 is E or V
  MISC_FEATURE (7)..(7): X at position 7 is A or E
  MISC_FEATURE (12)..(12): X at position 12 is A or E
LDQLLXXFIMMXL

SEQ ID NO: 291 - protein, 13 aa, Artificial
  Synthetic peptide
  MISC_FEATURE (6)..(6): X at position 6 is E or V
  MISC_FEATURE (10)..(10): X at position 10 is A or E
  MISC_FEATURE (11)..(11): X at position 11 is A or E
LDQLLXMFIXXML

SEQ ID NO: 292 - protein, 13 aa, Artificial
  Synthetic peptide
  MISC_FEATURE (6)..(6): X at position 6 is E or V
  MISC_FEATURE (10)..(10): X at position 10 is A or E
  MISC_FEATURE (12)..(12): X at position 12 is A or E
LDQLLXMFIXMXL

SEQ ID NO: 293 - protein, 13 aa, Artificial
  Synthetic peptide
  MISC_FEATURE (6)..(6): X at position 6 is E or V
  MISC_FEATURE (11)..(11): X at position 11 is A or E
  MISC_FEATURE (12)..(12): X at position 12 is A or E
LDQLLXMFIMXXL

SEQ ID NO: 294 - protein, 13 aa, Artificial
  Synthetic peptide
  MISC_FEATURE (6)..(6): X at position 6 is E or V
  MISC_FEATURE (10)..(10): X at position 10 is A or E
  MISC_FEATURE (11)..(11): X at position 11 is A or E
  MISC_FEATURE (12)..(12): X at position 12 is A or E
LDQLLXMFIXXXL

SEQ ID NO: 295 - protein, 15 aa, Artificial
  Synthetic peptide
  MISC_FEATURE (6)..(6): X at position 6 is E or V
  MISC_FEATURE (9)..(9): `X at position 9 is A or E
  MISC_FEATURE (13)..(13): `X at position 13 is A or E
  MISC_FEATURE (14)..(14): `X at position 14 is A or E
LDQLLXLLXFIMXXL

SEQ ID NO: 296 - protein, 15 aa, Artificial
  Synthetic peptide
  MISC_FEATURE (6)..(6): X at position 6 is E or V
  MISC_FEATURE (9)..(9): X at position 9 is A or E
  MISC_FEATURE (12)..(12): X at position 12 is A or E
  MISC_FEATURE (14)..(14): X at position 14 is A or E
LDQLLXLLXFIXMXL

SEQ ID NO: 297 - protein, 15 aa, Artificial
  Synthetic peptide
  MISC_FEATURE (6)..(6): X at position 6 is E or V
  MISC_FEATURE (9)..(9): X at position 9 is A or E
  MISC_FEATURE (12)..(12): X at position 12 is A or E
  MISC_FEATURE (13)..(13): X at position 13 is A or E
LDQLLXLLXFIXXML

SEQ ID NO: 298 - protein, 13 aa, Artificial
  Synthetic peptide
  MISC_FEATURE (6)..(6): X at position 6 is E or V
  MISC_FEATURE (7)..(7): X at position 7 is A or E
  MISC_FEATURE (10)..(10): X at position 10 is A or E
  MISC_FEATURE (11)..(11): X at position 11 is A or E
  MISC_FEATURE (12)..(12): X at position 12 is A or E
LDQLLXXFIXXXL

SEQ ID NO: 299 - protein, 12 aa, Artificial
  Synthetic peptide
  MISC_FEATURE (6)..(6): `X at position 6 is E or V
LDLLLXFIMMML

SEQ ID NO: 300 - protein, 12 aa, Artificial
  Synthetic peptide
  MISC_FEATURE (6)..(6): X at position 6 is E or V
  MISC_FEATURE (9)..(9): X at position 9 is A or E
LDLLLXFIXMML

SEQ ID NO: 301 - protein, 12 aa, Artificial
  Synthetic peptide
  MISC_FEATURE (6)..(6): X at position 6 is E or V
  MISC_FEATURE (10)..(10): X at position 10 is A or E
LDLLLXFIMXML

SEQ ID NO: 302 - protein, 12 aa, Artificial
  Synthetic peptide
  MISC_FEATURE (6)..(6): X at position 6 is E or V
  MISC_FEATURE (11)..(11): X at position 11 is A or E
LDLLLXFIMMXL

SEQ ID NO: 303 - protein, 12 aa, Artificial
  Synthetic peptide
  MISC_FEATURE (6)..(6): X at position 6 is E or V
  MISC_FEATURE (9)..(9): X at position 9 is A or E
  MISC_FEATURE (10)..(10): X at position 10 is A or E
LDLLLXFIXXML

SEQ ID NO: 304 - protein, 12 aa, Artificial
  Synthetic peptide
  MISC_FEATURE (6)..(6): X at position 6 is E or V
  MISC_FEATURE (9)..(9): X at position 9 is A or E
  MISC_FEATURE (11)..(11): X at position 11 is A or E
LDLLLXFIXMXL

SEQ ID NO: 305 - protein, 12 aa, Artificial
  Synthetic peptide
  MISC_FEATURE (6)..(6): X at position 6 is E or V
  MISC_FEATURE (10)..(10): X at position 10 is A or E
  MISC_FEATURE (11)..(11): X at position 11 is A or E
LDLLLXFIMXXL

SEQ ID NO: 306 - protein, 12 aa, Artificial
  Synthetic peptide
  MISC_FEATURE (6)..(6): X at position 6 is E or V
  MISC_FEATURE (9)..(9): X at position 9 is A or E
  MISC_FEATURE (10)..(10): X at position 10 is A or E
  MISC_FEATURE (11)..(11): X at position 11 is A or E
LDLLLXFIXXXL

SEQ ID NO: 307 - protein, 13 aa, Artificial
  Synthetic peptide
  MISC_FEATURE (7)..(7): X at position 7 is E or V
LDQLLLXFIMMML

SEQ ID NO: 308 - protein, 13 aa, Artificial
  Synthetic peptide
  MISC_FEATURE (7)..(7): X at position 7 is E or V
  MISC_FEATURE (10)..(10): X at position 10 is A or E
LDQLLLXFIXMML

SEQ ID NO: 309 - protein, 13 aa, Artificial
  Synthetic peptide
  MISC_FEATURE (7)..(7): X at position 7 is E or V
  MISC_FEATURE (11)..(11): X at position 11 is A or E
LDQLLLXFIMXML

SEQ ID NO: 310 - protein, 13 aa, Artificial
  Synthetic peptide
  MISC_FEATURE (7)..(7): X at position 7 is E or V
  MISC_FEATURE (12)..(12): X at position 12 is A or E
LDQLLLXFIMMXL

SEQ ID NO: 311 - protein, 13 aa, Artificial
  Synthetic peptide
  MISC_FEATURE (7)..(7): X at position 7 is E or V
  MISC_FEATURE (10)..(10): X at position 10 is A or E
  MISC_FEATURE (11)..(11): X at position 11 is A or E
LDQLLLXFIXXML

SEQ ID NO: 312 - protein, 13 aa, Artificial
  Synthetic peptide
  MISC_FEATURE (7)..(7): X at position 7 is E or V
  MISC_FEATURE (10)..(10): X at position 10 is A or E
  MISC_FEATURE (12)..(12): X at position 12 is A or E
LDQLLLXFIXMXL

SEQ ID NO: 313 - protein, 13 aa, Artificial
  Synthetic peptide
  MISC_FEATURE (7)..(7): X at position 7 is E or V
  MISC_FEATURE (11)..(11): X at position 11 is A or E
  MISC_FEATURE (12)..(12): X at position 12 is A or E
LDQLLLXFIMXXL

SEQ ID NO: 314 - protein, 13 aa, Artificial
  Synthetic peptide
  MISC_FEATURE (7)..(7): X at position 7 is E or V
  MISC_FEATURE (10)..(10): X at position 10 is A or E
  MISC_FEATURE (11)..(11): X at position 11 is A or E
  MISC_FEATURE (12)..(12): X at position 12 is A or E
LDQLLLXFIXXXL

SEQ ID NO: 315 - protein, 12 aa, Artificial
  Synthetic peptide
  MISC_FEATURE (7)..(7): X at position 7 is E or V
LDLLLMXIMMML

SEQ ID NO: 316 - protein, 12 aa, Artificial
  Synthetic peptide
  MISC_FEATURE (6)..(6): X at position 6 is A or E
  MISC_FEATURE (7)..(7): X at position 7 is E or V
LDLLLXXIMMML

SEQ ID NO: 317 - protein, 12 aa, Artificial
  Synthetic peptide
  MISC_FEATURE (7)..(7): X at position 7 is E or V
  MISC_FEATURE (9)..(9): X at position 9 is A or E
LDLLLMXIXMML

SEQ ID NO: 318 - protein, 12 aa, Artificial
  Synthetic peptide
  MISC_FEATURE (7)..(7): X at position 7 is E or V
  MISC_FEATURE (10)..(10): X at position 10 is A or E
LDLLLMXIMXML

SEQ ID NO: 319 - protein, 12 aa, Artificial
  Synthetic peptide
  MISC_FEATURE (7)..(7): X at position 7 is E or V
  MISC_FEATURE (11)..(11): X at position 11 is A or E
LDLLLMXIMMXL

SEQ ID NO: 320 - protein, 12 aa, Artificial
  Synthetic peptide
  MISC_FEATURE (6)..(6): X at position 6 is A or E
  MISC_FEATURE (7)..(7): X at position 7 is E or V
  MISC_FEATURE (9)..(9): X at position 9 is A or E
LDLLLXXIXMML

SEQ ID NO: 321 - protein, 12 aa, Artificial
  Synthetic peptide
  MISC_FEATURE (6)..(6): X at position 6 is A or E
  MISC_FEATURE (7)..(7): X at position 7 is E or V
  MISC_FEATURE (10)..(10): X at position 10 is A or E
LDLLLXXIMXML

SEQ ID NO: 322 - protein, 12 aa, Artificial
  Synthetic peptide
  MISC_FEATURE (6)..(6): X at position 6 is A or E
  MISC_FEATURE (7)..(7): X at position 7 is E or V
  MISC_FEATURE (11)..(11): X at position 11 is A or E
LDLLLXXIMMXL

SEQ ID NO: 323 - protein, 12 aa, Artificial
  Synthetic peptide
  MISC_FEATURE (7)..(7): X at position 7 is E or V
  MISC_FEATURE (9)..(9): X at position 9 is A or E
  MISC_FEATURE (10)..(10): X at position 10 is A or E
LDLLLMXIXXML

SEQ ID NO: 324 - protein, 12 aa, Artificial
  Synthetic peptide
  MISC_FEATURE (7)..(7): X at position 7 is E or V
  MISC_FEATURE (9)..(9): X at position 9 is A or E
  MISC_FEATURE (11)..(11): X at position 11 is A or E
LDLLLMXIXMXL

SEQ ID NO: 325 - protein, 12 aa, Artificial
  Synthetic peptide
  MISC_FEATURE (7)..(7): X at position 7 is E or V
  MISC_FEATURE (10)..(10): X at position 10 is A or E
  MISC_FEATURE (11)..(11): X at position 11 is A or E
LDLLLMXIMXXL

SEQ ID NO: 326 - protein, 12 aa, Artificial
  Synthetic peptide
  MISC_FEATURE (6)..(6): X at position 6 is A or E
  MISC_FEATURE (7)..(7): X at position 7 is E or V
  MISC_FEATURE (10)..(10): X at position 10 is A or E
  MISC_FEATURE (11)..(11): X at position 11 is A or E
LDLLLXXIMXXL

SEQ ID NO: 327 - protein, 12 aa, Artificial
  Synthetic peptide
  MISC_FEATURE (6)..(6): X at position 6 is A or E
  MISC_FEATURE (7)..(7): X at position 7 is E or V
  MISC_FEATURE (9)..(9): X at position 9 is A or E
  MISC_FEATURE (11)..(11): X at position 11 is A or E
LDLLLXXIXMXL

SEQ ID NO: 328 - protein, 12 aa, Artificial
  Synthetic peptide
  MISC_FEATURE (6)..(6): X at position 6 is A or E
  MISC_FEATURE (7)..(7): X at position 7 is E or V
  MISC_FEATURE (9)..(9): X at position 9 is A or E
  MISC_FEATURE (10)..(10): X at position 10 is A or E
LDLLLXXIXXML

SEQ ID NO: 329 - protein, 12 aa, Artificial
  Synthetic peptide
  MISC_FEATURE (7)..(7): X at position 7 is E or V
  MISC_FEATURE (9)..(9): X at position 9 is A or E
  MISC_FEATURE (10)..(10): X at position 10 is A or E
  MISC_FEATURE (11)..(11): X at position 11 is A or E
LDLLLMXIXXXL

SEQ ID NO: 330 - protein, 13 aa, Artificial
  Synthetic peptide
  MISC_FEATURE (8)..(8): X at position 8 is E or V
LDQLLLMXIMMML

SEQ ID NO: 331 - protein, 13 aa, Artificial
  Synthetic peptide
  MISC_FEATURE (7)..(7): X at position 7 is A or E
  MISC_FEATURE (8)..(8): X at position 8 is E or V
LDQLLLXXIMMML

SEQ ID NO: 332 - protein, 13 aa, Artificial
  Synthetic peptide
  MISC_FEATURE (8)..(8): X at position 8 is E or V
  MISC_FEATURE (10)..(10): X at position 10 is A or E
LDQLLLMXIXMML

SEQ ID NO: 333 - protein, 13 aa, Artificial
  Synthetic peptide
  MISC_FEATURE (8)..(8): X at position 8 is E or V
  MISC_FEATURE (11)..(11): X at position 11 is A or E
LDQLLLMXIMXML

SEQ ID NO: 334 - protein, 13 aa, Artificial
  Synthetic peptide
  MISC_FEATURE (8)..(8): X at position 8 is E or V
  MISC_FEATURE (12)..(12): X at position 12 is A or E
LDQLLLMXIMMXL

SEQ ID NO: 335 - protein, 13 aa, Artificial
  Synthetic peptide
  MISC_FEATURE (7)..(7): X at position 7 is A or E
  MISC_FEATURE (8)..(8): X at position 8 is E or V
  MISC_FEATURE (10)..(10): X at position 10 is A or E
LDQLLLXXIXMML

SEQ ID NO: 336 - protein, 13 aa, Artificial
  Synthetic peptide
  MISC_FEATURE (7)..(7): X at position 7 is A or E
  MISC_FEATURE (8)..(8): X at position 8 is E or V
  MISC_FEATURE (11)..(11): X at position 11 is A or E
LDQLLLXXIMXML

SEQ ID NO: 337 - protein, 13 aa, Artificial
  Synthetic peptide
  MISC_FEATURE (7)..(7): X at position 7 is A or E
  MISC_FEATURE (8)..(8): X at position 8 is E or V
  MISC_FEATURE (12)..(12): X at position 12 is A or E
LDQLLLXXIMMXL

SEQ ID NO: 338 - protein, 13 aa, Artificial
  Synthetic peptide
  MISC_FEATURE (8)..(8): X at position 8 is E or V
  MISC_FEATURE (10)..(10): X at position 10 is A or E
  MISC_FEATURE (11)..(11): X at position 11 is A or E
LDQLLLMXIXXML

SEQ ID NO: 339 - protein, 13 aa, Artificial
  Synthetic peptide
  MISC_FEATURE (8)..(8): X at position 8 is E or V
  MISC_FEATURE (10)..(10): X at position 10 is A or E
  MISC_FEATURE (12)..(12): X at position 12 is A or E
LDQLLLMXIXMXL

SEQ ID NO: 340 - protein, 13 aa, Artificial
  Synthetic peptide
  MISC_FEATURE (8)..(8): X at position 8 is E or V
  MISC_FEATURE (11)..(11): X at position 11 is A or E
  MISC_FEATURE (12)..(12): X at position 12 is A or E
LDQLLLMXIMXXL

SEQ ID NO: 341 - protein, 13 aa, Artificial
  Synthetic peptide
  MISC_FEATURE (7)..(7): X at position 7 is A or E
  MISC_FEATURE (8)..(8): X at position 8 is E or V
  MISC_FEATURE (11)..(11): X at position 11 is A or E
  MISC_FEATURE (12)..(12): X at position 12 is A or E
LDQLLLXXIMXXL

SEQ ID NO: 342 - protein, 13 aa, Artificial
  Synthetic peptide
  MISC_FEATURE (7)..(7): X at position 7 is A or E
  MISC_FEATURE (8)..(8): X at position 8 is E or V
  MISC_FEATURE (10)..(10): X at position 10 is A or E
  MISC_FEATURE (12)..(12): X at position 12 is A or E
LDQLLLXXIXMXL

SEQ ID NO: 343 - protein, 13 aa, Artificial
  Synthetic peptide
  MISC_FEATURE (7)..(7): X at position 7 is A or E
  MISC_FEATURE (8)..(8): X at position 8 is E or V
  MISC_FEATURE (10)..(10): X at position 10 is A or E
  MISC_FEATURE (11)..(11): X at position 11 is A or E
LDQLLLXXIXXML

SEQ ID NO: 344 - protein, 13 aa, Artificial
  Synthetic peptide
  MISC_FEATURE (8)..(8): X at position 8 is E or V
  MISC_FEATURE (10)..(10): X at position 10 is A or E
  MISC_FEATURE (11)..(11): X at position 11 is A or E
  MISC_FEATURE (12)..(12): X at position 12 is A or E
LDQLLLMXIXXXL

SEQ ID NO: 345 - protein, 12 aa, Artificial
  Synthetic peptide
  MISC_FEATURE (8)..(8): X at position 8 is E or V
LDLLLMFXMMML

SEQ ID NO: 346 - protein, 12 aa, Artificial
  Synthetic peptide
  MISC_FEATURE (6)..(6): X at position 6 is A or E
  MISC_FEATURE (8)..(8): X at position 8 is E or V
LDLLLXFXMMML

SEQ ID NO: 347 - protein, 12 aa, Artificial
  Synthetic peptide
  MISC_FEATURE (8)..(8): X at position 8 is E or V
  MISC_FEATURE (9)..(9): X at position 9 is A or E
LDLLLMFXXMML

SEQ ID NO: 348 - protein, 12 aa, Artificial
  Synthetic peptide
  MISC_FEATURE (8)..(8): X at position 8 is E or V
  MISC_FEATURE (10)..(10): X at position 10 is A or E
LDLLLMFXMXML

SEQ ID NO: 349 - protein, 12 aa, Artificial
  Synthetic peptide
  MISC_FEATURE (8)..(8): X at position 8 is E or V
  MISC_FEATURE (11)..(11): X at position 11 is A or E
LDLLLMFXMMXL

SEQ ID NO: 350 - protein, 12 aa, Artificial
  Synthetic peptide
  MISC_FEATURE (6)..(6): X at position 6 is A or E
  MISC_FEATURE (8)..(8): X at position 8 is E or V
  MISC_FEATURE (9)..(9): X at position 9 is A or E
LDLLLXFXXMML

SEQ ID NO: 351 - protein, 12 aa, Artificial
  Synthetic peptide
  MISC_FEATURE (6)..(6): X at position 6 is A or E
  MISC_FEATURE (8)..(8): X at position 8 is E or V
  MISC_FEATURE (10)..(10): X at position 10 is A or E
LDLLLXFXMXML

SEQ ID NO: 352 - protein, 12 aa, Artificial
  Synthetic peptide
  MISC_FEATURE (6)..(6): X at position 6 is A or E
  MISC_FEATURE (8)..(8): X at position 8 is E or V
  MISC_FEATURE (11)..(11): X at position 11 is A or E
LDLLLXFXMMXL

SEQ ID NO: 353 - protein, 12 aa, Artificial
  Synthetic peptide
  MISC_FEATURE (8)..(8): X at position 8 is E or V
  MISC_FEATURE (9)..(9): X at position 9 is A or E
  MISC_FEATURE (10)..(10): X at position 10 is A or E
LDLLLMFXXXML

SEQ ID NO: 354 - protein, 12 aa, Artificial
  Synthetic peptide
  MISC_FEATURE (8)..(8): X at position 8 is E or V
  MISC_FEATURE (9)..(9): X at position 9 is A or E
  MISC_FEATURE (11)..(11): X at position 11 is A or E
LDLLLMFXXMXL

SEQ ID NO: 355 - protein, 12 aa, Artificial
  Synthetic peptide
  MISC_FEATURE (8)..(8): X at position 8 is E or V
  MISC_FEATURE (10)..(10): X at position 10 is A or E
  MISC_FEATURE (11)..(11): X at position 11 is A or E
LDLLLMFXMXXL

SEQ ID NO: 356 - protein, 12 aa, Artificial
  Synthetic peptide
  MISC_FEATURE (8)..(8): X at position 8 is E or V
  MISC_FEATURE (9)..(9): X at position 9 is A or E
  MISC_FEATURE (10)..(10): X at position 10 is A or E
  MISC_FEATURE (11)..(11): X at position 11 is A or E
LDLLLMFXXXXL

SEQ ID NO: 357 - protein, 12 aa, Artificial
  Synthetic peptide
  MISC_FEATURE (6)..(6): X at position 6 is A or E
  MISC_FEATURE (8)..(8): X at position 8 is E or V
  MISC_FEATURE (10)..(10): X at position 10 is A or E
  MISC_FEATURE (11)..(11): X at position 11 is A or E
LDLLLXFXMXXL

SEQ ID NO: 358 - protein, 12 aa, Artificial
  Synthetic peptide
  MISC_FEATURE (6)..(6): X at position 6 is A or E
  MISC_FEATURE (8)..(8): X at position 8 is E or V
  MISC_FEATURE (9)..(9): X at position 9 is A or E
  MISC_FEATURE (11)..(11): X at position 11 is A or E
LDLLLXFXXMXL

SEQ ID NO: 359 - protein, 12 aa, Artificial
  Synthetic peptide
  MISC_FEATURE (6)..(6): X at position 6 is A or E
  MISC_FEATURE (8)..(8): X at position 8 is E or V
  MISC_FEATURE (9)..(9): X at position 9 is A or E
  MISC_FEATURE (10)..(10): X at position 10 is A or E
LDLLLXFXXXML

SEQ ID NO: 360 - protein, 12 aa, Artificial
  Synthetic peptide
  MISC_FEATURE (6)..(6): X at position 6 is A or E
  MISC_FEATURE (8)..(8): X at position 8 is E or V
  MISC_FEATURE (9)..(9): X at position 9 is A or E
  MISC_FEATURE (10)..(10): X at position 10 is A or E
  MISC_FEATURE (11)..(11): X at position 11 is A or E
LDLLLXFXXXXL

SEQ ID NO: 361 - protein, 13 aa, Artificial
  Synthetic peptide
  MISC_FEATURE (9)..(9): X at position 9 is E or V
LDQLLLMFXMMML

SEQ ID NO: 362 - protein, 13 aa, Artificial
  Synthetic peptide
  MISC_FEATURE (7)..(7): X at position 7 is A or E
  MISC_FEATURE (9)..(9): X at position 9 is E or V
LDQLLLXFXMMML

SEQ ID NO: 363 - protein, 13 aa, Artificial
  Synthetic peptide
  MISC_FEATURE (9)..(9): X at position 9 is E or V
  MISC_FEATURE (10)..(10): X at position 10 is A or E
LDQLLLMFXXMML

SEQ ID NO: 364 - protein, 13 aa, Artificial
  Synthetic peptide
  MISC_FEATURE (9)..(9): X at position 9 is E or V
  MISC_FEATURE (11)..(11): X at position 11 is A or E
LDQLLLMFXMXML

SEQ ID NO: 365 - protein, 13 aa, Artificial
  Synthetic peptide
  MISC_FEATURE (9)..(9): X at position 9 is E or V
  MISC_FEATURE (12)..(12): X at position 12 is A or E
LDQLLLMFXMMXL

SEQ ID NO: 366 - protein, 13 aa, Artificial
  Synthetic peptide
  MISC_FEATURE (7)..(7): X at position 7 is A or E
  MISC_FEATURE (9)..(9): X at position 9 is E or V
  MISC_FEATURE (10)..(10): X at position 10 is A or E
LDQLLLXFXXMML

SEQ ID NO: 367 - protein, 13 aa, Artificial
  Synthetic peptide
  MISC_FEATURE (7)..(7): X at position 7 is A or E
  MISC_FEATURE (9)..(9): X at position 9 is E or V
  MISC_FEATURE (11)..(11): X at position 11 is A or E
LDQLLLXFXMXML

SEQ ID NO: 368 - protein, 13 aa, Artificial
  Synthetic peptide
  MISC_FEATURE (7)..(7): X at position 7 is A or E
  MISC_FEATURE (9)..(9): X at position 9 is E or V
  MISC_FEATURE (12)..(12): X at position 12 is A or E
LDQLLLXFXMMXL

SEQ ID NO: 369 - protein, 13 aa, Artificial
  Synthetic peptide
  MISC_FEATURE (9)..(9): X at position 9 is E or V
  MISC_FEATURE (10)..(10): X at position 10 is A or E
  MISC_FEATURE (11)..(11): X at position 11 is A or E
LDQLLLMFXXXML

SEQ ID NO: 370 - protein, 13 aa, Artificial
  Synthetic peptide
  MISC_FEATURE (9)..(9): X at position 9 is E or V
  MISC_FEATURE (10)..(10): X at position 10 is A or E
  MISC_FEATURE (12)..(12): X at position 12 is A or E
LDQLLLMFXXMXL

SEQ ID NO: 371 - protein, 13 aa, Artificial
  Synthetic peptide
  MISC_FEATURE (9)..(9): X at position 9 is E or V
  MISC_FEATURE (11)..(11): X at position 11 is A or E
  MISC_FEATURE (12)..(12): X at position 12 is A or E
LDQLLLMFXMXXL

SEQ ID NO: 372 - protein, 13 aa, Artificial
  Synthetic peptide
  MISC_FEATURE (9)..(9): X at position 9 is E or V
  MISC_FEATURE (10)..(10): X at position 10 is A or E
  MISC_FEATURE (11)..(11): X at position 11 is A or E
  MISC_FEATURE (12)..(12): X at position 12 is A or E
LDQLLLMFXXXXL

SEQ ID NO: 373 - protein, 13 aa, Artificial
  Synthetic peptide
  MISC_FEATURE (7)..(7): X at position 7 is A or E
  MISC_FEATURE (9)..(9): X at position 9 is E or V
  MISC_FEATURE (11)..(11): X at position 11 is A or E
  MISC_FEATURE (12)..(12): X at position 12 is A or E
LDQLLLXFXMXXL

SEQ ID NO: 374 - protein, 13 aa, Artificial
  Synthetic peptide
  MISC_FEATURE (7)..(7): X at position 7 is A or E
  MISC_FEATURE (9)..(9): X at position 9 is E or V
  MISC_FEATURE (10)..(10): X at position 10 is A or E
  MISC_FEATURE (12)..(12): X at position 12 is A or E
LDQLLLXFXXMXL

SEQ ID NO: 375 - protein, 13 aa, Artificial
  Synthetic peptide
  MISC_FEATURE (7)..(7): X at position 7 is A or E
  MISC_FEATURE (9)..(9): X at position 9 is E or V
  MISC_FEATURE (10)..(10): X at position 10 is A or E
  MISC_FEATURE (11)..(11): X at position 11 is A or E
LDQLLLXFXXXML

SEQ ID NO: 376 - protein, 13 aa, Artificial
  Synthetic peptide
  MISC_FEATURE (7)..(7): X at position 7 is A or E
  MISC_FEATURE (9)..(9): X at position 9 is E or V
  MISC_FEATURE (10)..(10): X at position 10 is A or E
  MISC_FEATURE (11)..(11): X at position 11 is A or E
  MISC_FEATURE (12)..(12): X at position 12 is A or E
LDQLLLXFXXXXL

SEQ ID NO: 377 - protein, 12 aa, Artificial
  Synthetic peptide
  MISC_FEATURE (9)..(9): X at position 9 is E or V
LDLLLMFIXMML

SEQ ID NO: 378 - protein, 12 aa, Artificial
  Synthetic peptide
  MISC_FEATURE (6)..(6): X at position 6 is A or E
  MISC_FEATURE (9)..(9): X at position 9 is E or V
LDLLLXFIXMML

SEQ ID NO: 379 - protein, 12 aa, Artificial
  Synthetic peptide
  MISC_FEATURE (9)..(9): X at position 9 is E or V
  MISC_FEATURE (10)..(10): X at position 10 is A or E
LDLLLMFIXXML

SEQ ID NO: 380 - protein, 12 aa, Artificial
  Synthetic peptide
  MISC_FEATURE (9)..(9): X at position 9 is E or V
  MISC_FEATURE (11)..(11): X at position 11 is A or E
LDLLLMFIXMXL

SEQ ID NO: 381 - protein, 12 aa, Artificial
  Synthetic peptide
  MISC_FEATURE (6)..(6): X at position 6 is A or E
  MISC_FEATURE (9)..(9): X at position 9 is E or V
  MISC_FEATURE (10)..(10): X at position 10 is A or E
LDLLLXFIXXML

SEQ ID NO: 382 - protein, 12 aa, Artificial
  Synthetic peptide
  MISC_FEATURE (6)..(6): X at position 6 is A or E
  MISC_FEATURE (9)..(9): X at position 9 is E or V
  MISC_FEATURE (10)..(10): X at position 10 is A or E
LDLLLXFIXXML

SEQ ID NO: 383 - protein, 12 aa, Artificial
  Synthetic peptide
  MISC_FEATURE (6)..(6): X at position 6 is A or E
  MISC_FEATURE (9)..(9): X at position 9 is E or V
  MISC_FEATURE (11)..(11): X at position 11 is A or E
LDLLLXFIXMXL

SEQ ID NO: 384 - protein, 12 aa, Artificial
  Synthetic peptide
  MISC_FEATURE (9)..(9): X at position 9 is E or V
  MISC_FEATURE (10)..(10): X at position 10 is A or E
  MISC_FEATURE (11)..(11): X at position 11 is A or E
LDLLLMFIXXXL

SEQ ID NO: 385 - protein, 12 aa, Artificial
  Synthetic peptide
  MISC_FEATURE (6)..(6): X at position 6 is A or E
  MISC_FEATURE (9)..(9): X at position 9 is E or V
  MISC_FEATURE (10)..(10): X at position 10 is A or E
  MISC_FEATURE (11)..(11): X at position 11 is A or E
LDLLLXFIXXXL

SEQ ID NO: 386 - protein, 13 aa, Artificial
  Synthetic peptide
  MISC_FEATURE (10)..(10): X at position 10 is E or V
LDQLLLMFIXMML

SEQ ID NO: 387 - protein, 13 aa, Artificial
  Synthetic peptide
  MISC_FEATURE (7)..(7): X at position 7 is A or E
  MISC_FEATURE (10)..(10): X at position 10 is E or V
LDQLLLXFIXMML

SEQ ID NO: 388 - protein, 13 aa, Artificial
  Synthetic peptide
  MISC_FEATURE (10)..(10): X at position 10 is E or V
  MISC_FEATURE (11)..(11): X at position 11 is A or E
LDQLLLMFIXXML

SEQ ID NO: 389 - protein, 13 aa, Artificial
  Synthetic peptide
  MISC_FEATURE (10)..(10): X at position 10 is E or V
  MISC_FEATURE (12)..(12): X at position 12 is A or E
LDQLLLMFIXMXL

SEQ ID NO: 390 - protein, 13 aa, Artificial
  Synthetic peptide
  MISC_FEATURE (7)..(7): X at position 7 is A or E
  MISC_FEATURE (10)..(10): X at position 10 is E or V
  MISC_FEATURE (11)..(11): X at position 11 is A or E
LDQLLLXFIXXML

SEQ ID NO: 391 - protein, 13 aa, Artificial
  Synthetic peptide
  MISC_FEATURE (7)..(7): X at position 7 is A or E
  MISC_FEATURE (10)..(10): X at position 10 is E or V
  MISC_FEATURE (12)..(12): X at position 12 is A or E
LDQLLLXFIXMXL

SEQ ID NO: 392 - protein, 13 aa, Artificial
  Synthetic peptide
  MISC_FEATURE (10)..(10): X at position 10 is E or V
  MISC_FEATURE (11)..(11): X at position 11 is A or E
  MISC_FEATURE (12)..(12): X at position 12 is A or E
LDQLLLMFIXXXL

SEQ ID NO: 393 - protein, 13 aa, Artificial
  Synthetic peptide
  MISC_FEATURE (7)..(7): X at position 7 is A or E
  MISC_FEATURE (10)..(10): X at position 10 is E or V
  MISC_FEATURE (11)..(11): X at position 11 is A or E
  MISC_FEATURE (12)..(12): X at position 12 is A or E
LDQLLLXFIXXXL

SEQ ID NO: 394 - protein, 12 aa, Artificial
  Synthetic peptide
  MISC_FEATURE (10)..(10): X at position 10 is E or V
LDLLLMFIMXML

SEQ ID NO: 395 - protein, 12 aa, Artificial
  Synthetic peptide
  MISC_FEATURE (6)..(6): X at position 6 is A or E
  MISC_FEATURE (10)..(10): X at position 10 is E or V
LDLLLXFIMXML

SEQ ID NO: 396 - protein, 12 aa, Artificial
  Synthetic peptide
  MISC_FEATURE (10)..(10): X at position 10 is E or V
  MISC_FEATURE (11)..(11): X at position 11 is A or E
LDLLLMFIMXXL

SEQ ID NO: 397 - protein, 12 aa, Artificial
  Synthetic peptide
  MISC_FEATURE (9)..(9): X at position 9 is A or E
  MISC_FEATURE (10)..(10): X at position 10 is E or V
LDLLLMFIXXML

SEQ ID NO: 398 - protein, 12 aa, Artificial
  Synthetic peptide
  MISC_FEATURE (6)..(6): X at position 6 is A or E
  MISC_FEATURE (10)..(10): X at position 10 is E or V
  MISC_FEATURE (11)..(11): X at position 11 is A or E
LDLLLXFIMXXL

SEQ ID NO: 399 - protein, 12 aa, Artificial
  Synthetic peptide
  MISC_FEATURE (6)..(6): X at position 6 is A or E
  MISC_FEATURE (9)..(9): X at position 9 is A or E
  MISC_FEATURE (10)..(10): X at position 10 is E or V
LDLLLXFIXXML

SEQ ID NO: 400 - protein, 12 aa, Artificial
  Synthetic peptide
  MISC_FEATURE (9)..(9): X at position 9 is A or E
  MISC_FEATURE (10)..(10): X at position 10 is E or V
  MISC_FEATURE (11)..(11): X at position 11 is A or E
LDLLLMFIXXXL

SEQ ID NO: 401 - protein, 12 aa, Artificial
  Synthetic peptide
  MISC_FEATURE (6)..(6): X at position 6 is A or E
  MISC_FEATURE (9)..(9): X at position 9 is A or E
  MISC_FEATURE (10)..(10): X at position 10 is E or V
  MISC_FEATURE (11)..(11): X at position 11 is A or E
LDLLLXFIXXXL

SEQ ID NO: 402 - protein, 13 aa, Artificial
  Synthetic peptide
  MISC_FEATURE (11)..(11): X at position 11 is E or V
LDQLLLMFIMXML

SEQ ID NO: 403 - protein, 13 aa, Artificial
  Synthetic peptide
  MISC_FEATURE (7)..(7): X at position 7 is A or E
  MISC_FEATURE (11)..(11): X at position 11 is E or V
LDQLLLXFIMXML

SEQ ID NO: 404 - protein, 13 aa, Artificial
  Synthetic peptide
  MISC_FEATURE (11)..(11): X at position 11 is E or V
  MISC_FEATURE (12)..(12): X at position 12 is A or E
LDQLLLMFIMXXL

SEQ ID NO: 405 - protein, 13 aa, Artificial
  Synthetic peptide
  MISC_FEATURE (10)..(10): X at position 10 is A or E
  MISC_FEATURE (11)..(11): X at position 11 is E or V
LDQLLLMFIXXML

SEQ ID NO: 406 - protein, 13 aa, Artificial
  Synthetic peptide
  MISC_FEATURE (7)..(7): X at position 7 is A or E
  MISC_FEATURE (11)..(11): X at position 11 is E or V
  MISC_FEATURE (12)..(12): X at position 12 is A or E
LDQLLLXFIMXXL

SEQ ID NO: 407 - protein, 13 aa, Artificial
  Synthetic peptide
  MISC_FEATURE (7)..(7): X at position 7 is A or E
  MISC_FEATURE (10)..(10): X at position 10 is A or E
  MISC_FEATURE (11)..(11): X at position 11 is E or V
LDQLLLXFIXXML

SEQ ID NO: 408 - protein, 13 aa, Artificial
  Synthetic peptide
  MISC_FEATURE (10)..(10): X at position 10 is A or E
  MISC_FEATURE (11)..(11): X at position 11 is E or V
  MISC_FEATURE (12)..(12): X at position 12 is A or E
LDQLLLMFIXXXL

SEQ ID NO: 409 - protein, 13 aa, Artificial
  Synthetic peptide
  MISC_FEATURE (7)..(7): X at position 7 is A or E
  MISC_FEATURE (10)..(10): X at position 10 is A or E
  MISC_FEATURE (11)..(11): X at position 11 is E or V
  MISC_FEATURE (12)..(12): X at position 12 is A or E
LDQLLLXFIXXXL

SEQ ID NO: 410 - protein, 12 aa, Artificial
  Synthetic peptide
  MISC_FEATURE (11)..(11): X at position 11 is E or V
LDLLLMFIMMXL

SEQ ID NO: 411 - protein, 12 aa, Artificial
  Synthetic peptide
  MISC_FEATURE (6)..(6): X at position 6 is A or E
  MISC_FEATURE (11)..(11): X at position 11 is E or V
LDLLLXFIMMXL

SEQ ID NO: 412 - protein, 12 aa, Artificial
  Synthetic peptide
  MISC_FEATURE (9)..(9): X at position 9 is A or E
  MISC_FEATURE (11)..(11): X at position 11 is E or V
LDLLLMFIXMXL

SEQ ID NO: 413 - protein, 12 aa, Artificial
  Synthetic peptide
  MISC_FEATURE (10)..(10): X at position 10 is A or E
  MISC_FEATURE (11)..(11): X at position 11 is E or V
LDLLLMFIMXXL

SEQ ID NO: 414 - protein, 12 aa, Artificial
  Synthetic peptide
  MISC_FEATURE (6)..(6): X at position 6 is A or E
  MISC_FEATURE (9)..(9): X at position 9 is A or E
  MISC_FEATURE (11)..(11): X at position 11 is E or V
LDLLLXFIXMXL

SEQ ID NO: 415 - protein, 12 aa, Artificial
  Synthetic peptide
  MISC_FEATURE (6)..(6): X at position 6 is A or E
  MISC_FEATURE (10)..(10): X at position 10 is A or E
  MISC_FEATURE (11)..(11): X at position 11 is E or V
LDLLLXFIMXXL

SEQ ID NO: 416 - protein, 12 aa, Artificial
  Synthetic peptide
  MISC_FEATURE (9)..(9): X at position 9 is A or E
  MISC_FEATURE (10)..(10): X at position 10 is A or E
  MISC_FEATURE (11)..(11): X at position 11 is E or V
LDLLLMFIXXXL

SEQ ID NO: 417 - protein, 12 aa, Artificial
  Synthetic peptide
  MISC_FEATURE (6)..(6): X at position 6 is A or E
  MISC_FEATURE (9)..(9): X at position 9 is A or E
  MISC_FEATURE (10)..(10): X at position 10 is A or E
  MISC_FEATURE (11)..(11): X at position 11 is E or V
LDLLLXFIXXXL

SEQ ID NO: 418 - protein, 13 aa, Artificial
  Synthetic peptide
  MISC_FEATURE (12)..(12): X at position 12 is E or V
LDQLLLMFIMMXL

SEQ ID NO: 419 - protein, 13 aa, Artificial
  Synthetic peptide
  MISC_FEATURE (7)..(7): X at position 7 is A or E
  MISC_FEATURE (12)..(12): X at position 12 is E or V
LDQLLLXFIMMXL

SEQ ID NO: 420 - protein, 13 aa, Artificial
  Synthetic peptide
  MISC_FEATURE (10)..(10): X at position 10 is A or E
  MISC_FEATURE (12)..(12): X at position 12 is E or V
LDQLLLMFIXMXL

SEQ ID NO: 421 - protein, 13 aa, Artificial
  Synthetic peptide
  MISC_FEATURE (11)..(11): X at position 11 is A or E
  MISC_FEATURE (12)..(12): X at position 12 is E or V
LDQLLLMFIMXXL

SEQ ID NO: 422 - protein, 13 aa, Artificial
  Synthetic peptide
  MISC_FEATURE (7)..(7): X at position 7 is A or E
  MISC_FEATURE (10)..(10): X at position 10 is A or E
  MISC_FEATURE (12)..(12): X at position 12 is E or V
LDQLLLXFIXMXL

SEQ ID NO: 423 - protein, 13 aa, Artificial
  Synthetic peptide
  MISC_FEATURE (7)..(7): X at position 7 is A or E
  MISC_FEATURE (11)..(11): X at position 11 is A or E
  MISC_FEATURE (12)..(12): X at position 12 is E or V
LDQLLLXFIMXXL

SEQ ID NO: 424 - protein, 13 aa, Artificial
  Synthetic peptide
  MISC_FEATURE (10)..(10): X at position 10 is A or E
  MISC_FEATURE (11)..(11): X at position 11 is A or E
  MISC_FEATURE (12)..(12): X at position 12 is E or V
LDQLLLMFIXXXL

SEQ ID NO: 425 - protein, 13 aa, Artificial
  Synthetic peptide
  MISC_FEATURE (7)..(7): X at position 7 is A or E
  MISC_FEATURE (10)..(10): X at position 10 is A or E
  MISC_FEATURE (11)..(11): X at position 11 is A or E
  MISC_FEATURE (12)..(12): X at position 12 is E or V
LDQLLLXFIXXXL

SEQ ID NO: 426 - protein, 12 aa, Artificial
  Synthetic peptide
  MISC_FEATURE (12)..(12): X at position 12 is E or V
LDLLLMFIMMMX

SEQ ID NO: 427 - protein, 12 aa, Artificial
  Synthetic peptide
  MISC_FEATURE (6)..(6): X at position 6 is A or E
  MISC_FEATURE (12)..(12): X at position 12 is E or V
LDLLLXFIMMMX

SEQ ID NO: 428 - protein, 12 aa, Artificial
  Synthetic peptide
  MISC_FEATURE (9)..(9): X at position 9 is A or E
  MISC_FEATURE (12)..(12): X at position 12 is E or V
LDLLLMFIXMMX

SEQ ID NO: 429 - protein, 12 aa, Artificial
  Synthetic peptide
  MISC_FEATURE (10)..(10): X at position 10 is A or E
  MISC_FEATURE (12)..(12): X at position 12 is E or V
LDLLLMFIMXMX

SEQ ID NO: 430 - protein, 12 aa, Artificial
  Synthetic peptide
  MISC_FEATURE (11)..(11): X at position 11 is A or E
  MISC_FEATURE (12)..(12): X at position 12 is E or V
LDLLLMFIMMXX

SEQ ID NO: 431 - protein, 12 aa, Artificial
  Synthetic peptide
  MISC_FEATURE (6)..(6): X at position 6 is A or E
  MISC_FEATURE (9)..(9): X at position 9 is A or E
  MISC_FEATURE (12)..(12): X at position 12 is E or V
LDLLLXFIXMMX

SEQ ID NO: 432 - protein, 12 aa, Artificial
  Synthetic peptide
  MISC_FEATURE (6)..(6): X at position 6 is A or E
  MISC_FEATURE (10)..(10): X at position 10 is A or E
  MISC_FEATURE (12)..(12): X at position 12 is E or V
LDLLLXFIMXMX

SEQ ID NO: 433 - protein, 12 aa, Artificial
  Synthetic peptide
  MISC_FEATURE (6)..(6): X at position 6 is A or E
  MISC_FEATURE (11)..(11): X at position 11 is A or E
  MISC_FEATURE (12)..(12): X at position 12 is E or V
LDLLLXFIMMXX

SEQ ID NO: 434 - protein, 12 aa, Artificial
  Synthetic peptide
  MISC_FEATURE (9)..(9): X at position 9 is A or E
  MISC_FEATURE (10)..(10): X at position 10 is A or E
  MISC_FEATURE (12)..(12): X at position 12 is E or V
LDLLLMFIXXMX

SEQ ID NO: 435 - protein, 12 aa, Artificial
  Synthetic peptide
  MISC_FEATURE (9)..(9): X at position 9 is A or E
  MISC_FEATURE (11)..(11): X at position 11 is A or E
  MISC_FEATURE (12)..(12): X at position 12 is E or V
LDLLLMFIXMXX

SEQ ID NO: 436 - protein, 12 aa, Artificial
  Synthetic peptide
  MISC_FEATURE (10)..(10): X at position 10 is A or E
  MISC_FEATURE (11)..(11): X at position 11 is A or E
  MISC_FEATURE (12)..(12): X at position 12 is E or V
LDLLLMFIMXXX

SEQ ID NO: 437 - protein, 12 aa, Artificial
  Synthetic peptide
  MISC_FEATURE (9)..(9): X at position 9 is A or E
  MISC_FEATURE (10)..(10): X at position 10 is A or E
  MISC_FEATURE (11)..(11): X at position 11 is A or E
  MISC_FEATURE (12)..(12): X at position 12 is E or V
LDLLLMFIXXXX

SEQ ID NO: 438 - protein, 12 aa, Artificial
  Synthetic peptide
  MISC_FEATURE (6)..(6): X at position 6 is A or E
  MISC_FEATURE (10)..(10): X at position 10 is A or E
  MISC_FEATURE (11)..(11): X at position 11 is A or E
  MISC_FEATURE (12)..(12): X at position 12 is E or V
LDLLLXFIMXXX

SEQ ID NO: 439 - protein, 12 aa, Artificial
  Synthetic peptide
  MISC_FEATURE (6)..(6): X at position 6 is A or E
  MISC_FEATURE (9)..(9): X at position 9 is A or E
  MISC_FEATURE (11)..(11): X at position 11 is A or E
  MISC_FEATURE (12)..(12): X at position 12 is E or V
LDLLLXFIXMXX

SEQ ID NO: 440 - protein, 12 aa, Artificial
  Synthetic peptide
  MISC_FEATURE (6)..(6): X at position 6 is A or E
  MISC_FEATURE (9)..(9): X at position 9 is A or E
  MISC_FEATURE (10)..(10): X at position 10 is A or E
  MISC_FEATURE (12)..(12): X at position 12 is E or V
LDLLLXFIXXMX

SEQ ID NO: 441 - protein, 12 aa, Artificial
  Synthetic peptide
  MISC_FEATURE (6)..(6): X at position 6 is A or E
  MISC_FEATURE (9)..(9): X at position 9 is A or E
  MISC_FEATURE (10)..(10): X at position 10 is A or E
  MISC_FEATURE (11)..(11): X at position 11 is A or E
  MISC_FEATURE (12)..(12): X at position 12 is E or V
LDLLLXFIXXXX

SEQ ID NO: 442 - protein, 13 aa, Artificial
  Synthetic peptide
  MISC_FEATURE (13)..(13): X at position 13 is E or V
LDQLLLMFIMMMX

SEQ ID NO: 443 - protein, 13 aa, Artificial
  Synthetic peptide
  MISC_FEATURE (7)..(7): X at position 7 is A or E
  MISC_FEATURE (13)..(13): X at position 13 is E or V
LDQLLLXFIMMMX

SEQ ID NO: 444 - protein, 13 aa, Artificial
  Synthetic peptide
  MISC_FEATURE (10)..(10): X at position 10 is A or E
  MISC_FEATURE (13)..(13): X at position 13 is E or V
LDQLLLMFIXMMX

SEQ ID NO: 445 - protein, 13 aa, Artificial
  Synthetic peptide
  MISC_FEATURE (11)..(11): X at position 11 is A or E
  MISC_FEATURE (13)..(13): X at position 13 is E or V
LDQLLLMFIMXMX

SEQ ID NO: 446 - protein, 13 aa, Artificial
  Synthetic peptide
  MISC_FEATURE (12)..(12): X at position 12 is A or E
  MISC_FEATURE (13)..(13): X at position 13 is E or V
LDQLLLMFIMMXX

SEQ ID NO: 447 - protein, 13 aa, Artificial
  Synthetic peptide
  MISC_FEATURE (7)..(7): X at position 7 is A or E
  MISC_FEATURE (10)..(10): X at position 10 is A or E
  MISC_FEATURE (13)..(13): X at position 13 is E or V
LDQLLLXFIXMMX

SEQ ID NO: 448 - protein, 13 aa, Artificial
  Synthetic peptide
  MISC_FEATURE (7)..(7): X at position 7 is A or E
  MISC_FEATURE (11)..(11): X at position 11 is A or E
  MISC_FEATURE (13)..(13): X at position 13 is E or V
LDQLLLXFIMXMX

SEQ ID NO: 449 - protein, 13 aa, Artificial
  Synthetic peptide
  MISC_FEATURE (7)..(7): X at position 7 is A or E
  MISC_FEATURE (12)..(12): X at position 12 is A or E
  MISC_FEATURE (13)..(13): X at position 13 is E or V
LDQLLLXFIMMXX

SEQ ID NO: 450 - protein, 13 aa, Artificial
  Synthetic peptide
  MISC_FEATURE (10)..(10): X at position 10 is A or E
  MISC_FEATURE (11)..(11): X at position 11 is A or E
  MISC_FEATURE (13)..(13): X at position 13 is E or V
LDQLLLMFIXXMX

SEQ ID NO: 451 - protein, 13 aa, Artificial
  Synthetic peptide
  MISC_FEATURE (10)..(10): X at position 10 is A or E
  MISC_FEATURE (12)..(12): X at position 12 is A or E
  MISC_FEATURE (13)..(13): X at position 13 is E or V
LDQLLLMFIXMXX

SEQ ID NO: 452 - protein, 13 aa, Artificial
  Synthetic peptide
  MISC_FEATURE (11)..(11): X at position 11 is A or E
  MISC_FEATURE (12)..(12): X at position 12 is A or E
  MISC_FEATURE (13)..(13): X at position 13 is E or V
LDQLLLMFIMXXX

SEQ ID NO: 453 - protein, 13 aa, Artificial
  Synthetic peptide
  MISC_FEATURE (10)..(10): X at position 10 is A or E
  MISC_FEATURE (11)..(11): X at position 11 is A or E
  MISC_FEATURE (12)..(12): X at position 12 is A or E
  MISC_FEATURE (13)..(13): X at position 13 is E or V
LDQLLLMFIXXXX

SEQ ID NO: 454 - protein, 13 aa, Artificial
  Synthetic peptide
  MISC_FEATURE (7)..(7): X at position 7 is A or E
  MISC_FEATURE (11)..(11): X at position 11 is A or E
  MISC_FEATURE (12)..(12): X at position 12 is A or E
  MISC_FEATURE (13)..(13): X at position 13 is E or V
LDQLLLXFIMXXX

SEQ ID NO: 455 - protein, 13 aa, Artificial
  Synthetic peptide
  MISC_FEATURE (7)..(7): X at position 7 is A or E
  MISC_FEATURE (10)..(10): X at position 10 is A or E
  MISC_FEATURE (12)..(12): X at position 12 is A or E
  MISC_FEATURE (13)..(13): X at position 13 is E or V
LDQLLLXFIXMXX

SEQ ID NO: 456 - protein, 13 aa, Artificial
  Synthetic peptide
  MISC_FEATURE (7)..(7): X at position 7 is A or E
  MISC_FEATURE (10)..(10): X at position 10 is A or E
  MISC_FEATURE (11)..(11): X at position 11 is A or E
  MISC_FEATURE (13)..(13): X at position 13 is E or V
LDQLLLXFIXXMX

SEQ ID NO: 457 - protein, 13 aa, Artificial
  Synthetic peptide
  MISC_FEATURE (7)..(7): X at position 7 is A or E
  MISC_FEATURE (10)..(10): X at position 10 is A or E
  MISC_FEATURE (11)..(11): X at position 11 is A or E
  MISC_FEATURE (12)..(12): X at position 12 is A or E
  MISC_FEATURE (13)..(13): X at position 13 is E or V
LDQLLLXFIXXXX

SEQ ID NO: 458 - protein, 12 aa, Artificial
  Synthetic peptide
LKLLLMFIMMML

SEQ ID NO: 459 - protein, 12 aa, Artificial
  Synthetic peptide
  MISC_FEATURE (6)..(6): X at position 6 is A or E
LKLLLXFIMMML

SEQ ID NO: 460 - protein, 12 aa, Artificial
  Synthetic peptide
  MISC_FEATURE (9)..(9): X at position 9 is A or E
LKLLLMFIXMML

SEQ ID NO: 461 - protein, 12 aa, Artificial
  Synthetic peptide
  MISC_FEATURE (10)..(10): X at position 10 is A or E
LKLLLMFIMXML

SEQ ID NO: 462 - protein, 12 aa, Artificial
  Synthetic peptide
  MISC_FEATURE (11)..(11): X at position 11 is A or E
LKLLLMFIMMXL

SEQ ID NO: 463 - protein, 12 aa, Artificial
  Synthetic peptide
  MISC_FEATURE (6)..(6): X at position 6 is A or E
  MISC_FEATURE (9)..(9): X at position 9 is A or E
LKLLLXFIXMML

SEQ ID NO: 464 - protein, 12 aa, Artificial
  Synthetic peptide
  MISC_FEATURE (6)..(6): X at position 6 is A or E
  MISC_FEATURE (10)..(10): X at position 10 is A or E
LKLLLXFIMXML

SEQ ID NO: 465 - protein, 12 aa, Artificial
  Synthetic peptide
  MISC_FEATURE (6)..(6): X at position 6 is A or E
  MISC_FEATURE (11)..(11): X at position 11 is A or E
LKLLLXFIMMXL

SEQ ID NO: 466 - protein, 12 aa, Artificial
  Synthetic peptide
  MISC_FEATURE (9)..(9): X at position 9 is A or E
  MISC_FEATURE (10)..(10): X at position 10 is A or E
LKLLLMFIXXML

SEQ ID NO: 467 - protein, 12 aa, Artificial
  Synthetic peptide
  MISC_FEATURE (9)..(9): X at position 9 is A or E
  MISC_FEATURE (11)..(11): X at position 11 is A or E
LKLLLMFIXMXL

SEQ ID NO: 468 - protein, 12 aa, Artificial
  Synthetic peptide
  MISC_FEATURE (10)..(10): X at position 10 is A or E
  MISC_FEATURE (11)..(11): X at position 11 is A or E
LKLLLMFIMXXL

SEQ ID NO: 469 - protein, 12 aa, Artificial
  Synthetic peptide
  MISC_FEATURE (9)..(9): X at position 9 is A or E
  MISC_FEATURE (10)..(10): X at position 10 is A or E
  MISC_FEATURE (11)..(11): X at position 11 is A or E
LKLLLMFIXXXL

SEQ ID NO: 470 - protein, 12 aa, Artificial
  Synthetic peptide
  MISC_FEATURE (6)..(6): X at position 6 is A or E
  MISC_FEATURE (10)..(10): X at position 10 is A or E
  MISC_FEATURE (11)..(11): X at position 11 is A or E
  MISC_FEATURE (12)..(12): X at position 12 is E or V
LKLLLXFIMXXX

SEQ ID NO: 471 - protein, 12 aa, Artificial
  Synthetic peptide
  MISC_FEATURE (6)..(6): X at position 6 is A or E
  MISC_FEATURE (9)..(9): X at position 9 is A or E
  MISC_FEATURE (11)..(11): X at position 11 is A or E
  MISC_FEATURE (12)..(12): X at position 12 is E or V
LKLLLXFIXMXX

SEQ ID NO: 472 - protein, 12 aa, Artificial
  Synthetic peptide
  MISC_FEATURE (6)..(6): X at position 6 is A or E
  MISC_FEATURE (9)..(9): X at position 9 is A or E
  MISC_FEATURE (10)..(10): X at position 10 is A or E
  MISC_FEATURE (12)..(12): X at position 12 is E or V
LKLLLXFIXXMX

SEQ ID NO: 473 - protein, 12 aa, Artificial
  Synthetic peptide
  MISC_FEATURE (6)..(6): X at position 6 is A or E
  MISC_FEATURE (9)..(9): X at position 9 is A or E
  MISC_FEATURE (10)..(10): X at position 10 is A or E
  MISC_FEATURE (11)..(11): X at position 11 is A or E
LKLLLXFIXXXL

SEQ ID NO: 474 - protein, 13 aa, Artificial
  Synthetic peptide
LKQLLLMFIMMML

SEQ ID NO: 475 - protein, 13 aa, Artificial
  Synthetic peptide
  MISC_FEATURE (7)..(7): X at position 7 is A or E
LKQLLLXFIMMML

SEQ ID NO: 476 - protein, 13 aa, Artificial
  Synthetic peptide
  MISC_FEATURE (10)..(10): X at position 10 is A or E
LKQLLLMFIXMML

SEQ ID NO: 477 - protein, 13 aa, Artificial
  Synthetic peptide
  MISC_FEATURE (11)..(11): X at position 11 is A or E
LKQLLLMFIMXML

SEQ ID NO: 478 - protein, 13 aa, Artificial
  Synthetic peptide
  MISC_FEATURE (12)..(12): X at position 12 is A or E
LKQLLLMFIMMXL

SEQ ID NO: 479 - protein, 13 aa, Artificial
  Synthetic peptide
  MISC_FEATURE (7)..(7): X at position 7 is A or E
  MISC_FEATURE (10)..(10): X at position 10 is A or E
LKQLLLXFIXMML

SEQ ID NO: 480 - protein, 13 aa, Artificial
  Synthetic peptide
  MISC_FEATURE (7)..(7): X at position 7 is A or E
  MISC_FEATURE (11)..(11): X at position 11 is A or E
LKQLLLXFIMXML

SEQ ID NO: 481 - protein, 13 aa, Artificial
  Synthetic peptide
  MISC_FEATURE (7)..(7): X at position 7 is A or E
  MISC_FEATURE (12)..(12): X at position 12 is A or E
LKQLLLXFIMMXL

SEQ ID NO: 482 - protein, 13 aa, Artificial
  Synthetic peptide
  MISC_FEATURE (10)..(10): X at position 10 is A or E
  MISC_FEATURE (11)..(11): X at position 11 is A or E
LKQLLLMFIXXML

SEQ ID NO: 483 - protein, 13 aa, Artificial
  Synthetic peptide
  MISC_FEATURE (10)..(10): X at position 10 is A or E
  MISC_FEATURE (12)..(12): X at position 12 is A or E
LKQLLLMFIXMXL

SEQ ID NO: 484 - protein, 13 aa, Artificial
  Synthetic peptide
  MISC_FEATURE (11)..(11): X at position 11 is A or E
  MISC_FEATURE (12)..(12): X at position 12 is A or E
LKQLLLMFIMXXL

SEQ ID NO: 485 - protein, 13 aa, Artificial
  Synthetic peptide
  MISC_FEATURE (10)..(10): X at position 10 is A or E
  MISC_FEATURE (11)..(11): X at position 11 is A or E
  MISC_FEATURE (12)..(12): X at position 12 is A or E
LKQLLLMFIXXXL

SEQ ID NO: 486 - protein, 13 aa, Artificial
  Synthetic peptide
  MISC_FEATURE (7)..(7): X at position 7 is A or E
  MISC_FEATURE (11)..(11): X at position 11 is A or E
  MISC_FEATURE (12)..(12): X at position 12 is A or E
  MISC_FEATURE (13)..(13): X at position 13 is E or V
LKQLLLXFIMXXX

SEQ ID NO: 487 - protein, 13 aa, Artificial
  Synthetic peptide
  MISC_FEATURE (7)..(7): X at position 7 is A or E
  MISC_FEATURE (10)..(10): X at position 10 is A or E
  MISC_FEATURE (12)..(12): X at position 12 is A or E
  MISC_FEATURE (13)..(13): X at position 13 is E or V
LKQLLLXFIXMXX

SEQ ID NO: 488 - protein, 13 aa, Artificial
  Synthetic peptide
  MISC_FEATURE (7)..(7): X at position 7 is A or E
  MISC_FEATURE (10)..(10): X at position 10 is A or E
  MISC_FEATURE (11)..(11): X at position 11 is A or E
  MISC_FEATURE (13)..(13): X at position 13 is E or V
LKQLLLXFIXXMX

SEQ ID NO: 489 - protein, 13 aa, Artificial
  Synthetic peptide
  MISC_FEATURE (7)..(7): X at position 7 is A or E
  MISC_FEATURE (10)..(10): X at position 10 is A or E
  MISC_FEATURE (11)..(11): X at position 11 is A or E
  MISC_FEATURE (12)..(12): X at position 12 is A or E
LKQLLLXFIXXXL

SEQ ID NO: 490 - protein, 13 aa, Artificial
  Synthetic peptide
  MISC_FEATURE (3)..(3): X at position 3 is E, S, or A
LDXLLLMFIMMML

SEQ ID NO: 491 - protein, 13 aa, Artificial
  Synthetic peptide
  MISC_FEATURE (3)..(3): X at position 3 is E, S, or A
  MISC_FEATURE (7)..(7): X at position 7 is A or E
LDXLLLXFIMMML

SEQ ID NO: 492 - protein, 13 aa, Artificial
  Synthetic peptide
  MISC_FEATURE (3)..(3): X at position 3 is E, S, or A
  MISC_FEATURE (10)..(10): X at position 10 is A or E
LDXLLLMFIXMML

SEQ ID NO: 493 - protein, 13 aa, Artificial
  Synthetic peptide
  MISC_FEATURE (3)..(3): X at position 3 is E, S, or A
  MISC_FEATURE (11)..(11): X at position 11 is A or E
LDXLLLMFIMXML

SEQ ID NO: 494 - protein, 13 aa, Artificial
  Synthetic peptide
  MISC_FEATURE (3)..(3): X at position 3 is E, S, or A
  MISC_FEATURE (12)..(12): X at position 12 is A or E
LDXLLLMFIMMXL

SEQ ID NO: 495 - protein, 13 aa, Artificial
  Synthetic peptide
  MISC_FEATURE (3)..(3): X at position 3 is E, S, or A
  MISC_FEATURE (7)..(7): X at position 7 is A or E
  MISC_FEATURE (10)..(10): X at position 10 is A or E
LDXLLLXFIXMML

SEQ ID NO: 496 - protein, 13 aa, Artificial
  Synthetic peptide
  MISC_FEATURE (3)..(3): X at position 3 is E, S, or A
  MISC_FEATURE (7)..(7): X at position 7 is A or E
  MISC_FEATURE (11)..(11): X at position 11 is A or E
LDXLLLXFIMXML

SEQ ID NO: 497 - protein, 13 aa, Artificial
  Synthetic peptide
  MISC_FEATURE (3)..(3): X at position 3 is E, S, or A
  MISC_FEATURE (7)..(7): X at position 7 is A or E
  MISC_FEATURE (12)..(12): X at position 12 is A or E
LDXLLLXFIMMXL

SEQ ID NO: 498 - protein, 13 aa, Artificial
  Synthetic peptide
  MISC_FEATURE (3)..(3): X at position 3 is E, S, or A
  MISC_FEATURE (10)..(10): X at position 10 is A or E
  MISC_FEATURE (11)..(11): X at position 11 is A or E
LDXLLLMFIXXML

SEQ ID NO: 499 - protein, 13 aa, Artificial
  Synthetic peptide
  MISC_FEATURE (3)..(3): X at position 3 is E, S, or A
  MISC_FEATURE (10)..(10): X at position 10 is A or E
  MISC_FEATURE (12)..(12): X at position 12 is A or E
LDXLLLMFIXMXL

SEQ ID NO: 500 - protein, 13 aa, Artificial
  Synthetic peptide
  MISC_FEATURE (3)..(3): X at position 3 is E, S, or A
  MISC_FEATURE (11)..(11): X at position 11 is A or E
  MISC_FEATURE (12)..(12): X at position 12 is A or E
LDXLLLMFIMXXL

SEQ ID NO: 501 - protein, 13 aa, Artificial
  Synthetic peptide
  MISC_FEATURE (3)..(3): X at position 3 is E, S, or A
  MISC_FEATURE (10)..(10): X at position 10 is A or E
  MISC_FEATURE (11)..(11): X at position 11 is A or E
  MISC_FEATURE (12)..(12): X at position 12 is A or E
LDXLLLMFIXXXL

SEQ ID NO: 502 - protein, 13 aa, Artificial
  Synthetic peptide
  MISC_FEATURE (3)..(3): X at position 3 is E, S, or A
  MISC_FEATURE (7)..(7): X at position 7 is A or E
  MISC_FEATURE (11)..(11): X at position 11 is A or E
  MISC_FEATURE (12)..(12): X at position 12 is A or E
LDXLLLXFIMXXL

SEQ ID NO: 503 - protein, 13 aa, Artificial
  Synthetic peptide
  MISC_FEATURE (3)..(3): X at position 3 is E, S, or A
  MISC_FEATURE (7)..(7): X at position 7 is A or E
  MISC_FEATURE (10)..(10): X at position 10 is A or E
  MISC_FEATURE (12)..(12): X at position 12 is A or E
LDXLLLXFIXMXL

SEQ ID NO: 504 - protein, 13 aa, Artificial
  Synthetic peptide
  MISC_FEATURE (3)..(3): X at position 3 is E, S, or A
  MISC_FEATURE (7)..(7): X at position 7 is A or E
  MISC_FEATURE (10)..(10): X at position 10 is A or E
  MISC_FEATURE (11)..(11): X at position 11 is A or E
LDXLLLXFIXXML

SEQ ID NO: 505 - protein, 13 aa, Artificial
  Synthetic peptide
  MISC_FEATURE (3)..(3): X at position 3 is E, S, or A
  MISC_FEATURE (7)..(7): X at position 7 is A or E
  MISC_FEATURE (10)..(10): X at position 10 is A or E
  MISC_FEATURE (11)..(11): X at position 11 is A or E
  MISC_FEATURE (12)..(12): X at position 12 is A or E
LDXLLLXFIXXXL

SEQ ID NO: 506 - DNA, 63 bp, Artificial
  P5 in E. coli
agcgcaggtagcgaacagcagctggatctgctgctgatgtttattatgatgatgctgcagcag

SEQ ID NO: 507 - DNA, 60 bp, Artificial
  P5-21 in E. coli
agcgaagaacagctggaactgctgctggcatttattgcagcagcactgcagcaggaagaa

SEQ ID NO: 508 - DNA, 63 bp, Artificial
  P5 in Zea mays
tccgccggctccgagcagcagctggacctgctgctgatgttcatcatgatgatgctgcagcag

SEQ ID NO: 509 - DNA, 60 bp, Artificial
  P5-21 in Zea mays
tccgaggagcagctggagctgctgctggccttcatcgccgccgccctgcagcaggaggag

SEQ ID NO: 510 - protein, 21 aa, Artificial
  Synthetic peptide
SAGSEQQEDLLLAFIAAALQQ

SEQ ID NO: 511 - protein, 21 aa, Artificial
  Synthetic peptide
SAGSEQQLDELLAFIAAALQQ

SEQ ID NO: 512 - protein, 21 aa, Artificial
  Synthetic peptide
SAGSEQQEDELLAFIAAALQQ

SEQ ID NO: 513 - protein, 21 aa, Artificial
  Synthetic peptide
SAGSEQQEDELLMFIMMMLQQ

SEQ ID NO: 514 - protein, 20 aa, Artificial
  Synthetic peptide
SEEQEELLLAFIAAALQQEE

SEQ ID NO: 515 - protein, 20 aa, Artificial
  Synthetic peptide
SEEQLEELLAFIAAALQQEE

SEQ ID NO: 516 - protein, 20 aa, Artificial
  Synthetic peptide
SEEQEEELLAFIAAALQQEE

SEQ ID NO: 517 - protein, 22 aa, Artificial
  Synthetic peptide
SAGSEQQLDLLLMFIMMMLQQR

SEQ ID NO: 518 - protein, 21 aa, Artificial
  Synthetic peptide
SEEQLELLLAFIAAALQQEER

SEQ ID NO: 519 - protein, 19 aa, Artificial
  Synthetic peptide
SAGSEQQEDLLLAFIALQQ

SEQ ID NO: 520 - protein, 19 aa, Artificial
  Synthetic peptide
SAGSEQQLDELLAFIALQQ

SEQ ID NO: 521 - protein, 19 aa, Artificial
  Synthetic peptide
SAGSEQQLDLLLEFIALQQ

SEQ ID NO: 522 - protein, 19 aa, Artificial
  Synthetic peptide
SAGSEQQLDLLLAEIALQQ

SEQ ID NO: 523 - protein, 20 aa, Artificial
  Synthetic peptide
SAGSEQQLDLLLAFIEALQQ

SEQ ID NO: 524 - protein, 21 aa, Artificial
  Synthetic peptide
SAGSEQQLDLLLAFIAEALQQ

SEQ ID NO: 525 - protein, 21 aa, Artificial
  Synthetic peptide
SAGSEQQLDLLLAFIEAALQQ

SEQ ID NO: 526 - protein, 21 aa, Artificial
  Synthetic peptide
SAGSEQQLDLLLAFIAAELQQ

SEQ ID NO: 527 - protein, 21 aa, Artificial
  Synthetic peptide
SAGSEQQLDLLLAEIAAALQQ

SEQ ID NO: 528 - protein, 21 aa, Artificial
  Synthetic peptide
SAGSEQQLDLLLEFIAAALQQ

SEQ ID NO: 529 - protein, 21 aa, Artificial
  Synthetic peptide
SAGSEQQEDLLLAFIAAALQQ

SEQ ID NO: 530 - protein, 21 aa, Artificial
  Synthetic peptide
SAGSEQQLDELLAFIAAALQQ

SEQ ID NO: 531 - protein, 21 aa, Artificial
  Synthetic peptide
SQAGSEQLDLLLMFIMMMLQQ

SEQ ID NO: 532 - protein, 21 aa, Artificial
  Synthetic peptide
AEQGSSQLDLLLMFIMMMLQQ

SEQ ID NO: 533 - protein, 23 aa, Artificial
  Synthetic peptide
NQGISEKQQLDLLLMFIMMMLQQ

SEQ ID NO: 534 - protein, 23 aa, Artificial
  Synthetic peptide
NQGISEKQQLDLLLAFIAAALQQ

SEQ ID NO: 535 - protein, 34 aa, Artificial
  Synthetic peptide
NFGTPDSTVQNPQDASKPNQLDLLLMFIMMMLQQ

SEQ ID NO: 536 - protein, 34 aa, Artificial
  Synthetic peptide
NFGTPDSTVQNPQDASKPNQLDLLLAFIAAALQQ

SEQ ID NO: 537 - protein, 30 aa, Artificial
  Synthetic peptide
ITPDGQGGGQIGDNPQLDLLLMFIMMMLQQ

SEQ ID NO: 538 - protein, 30 aa, Artificial
  Synthetic peptide
ITPDGQGGGQIGDNPQLDLLLAFIAAALQQ

SEQ ID NO: 539 - protein, 20 aa, Artificial
  Synthetic peptide
SEEQLDLLLAFIAAALQQEE

SEQ ID NO: 540 - protein, 19 aa, Artificial
  Synthetic peptide
SEEQLELLLAFIAAALQEE

SEQ ID NO: 541 - protein, 21 aa, Artificial
  Synthetic peptide
SAGSEEELDLLLMFIMMMLQQ

SEQ ID NO: 542 - protein, 21 aa, Artificial
  Synthetic peptide
SAGSEQQLDLLLMFIMMMLEE

SEQ ID NO: 543 - protein, 21 aa, Artificial
  Synthetic peptide
SEEQQLDLLLMFIMMMLQQEE

SEQ ID NO: 544 - protein, 22 aa, Artificial
  Synthetic peptide
SEEEEQLDQLLLAFIAAALQQR

SEQ ID NO: 545 - protein, 15 aa, Artificial
  Synthetic peptide
QLEQLLAFIAAALQQ

SEQ ID NO: 546 - protein, 15 aa, Artificial
  Synthetic peptide
QLDLLLAFIAAALQQ

SEQ ID NO: 547 - protein, 5 aa, Artificial
  Enterokinase cleavage site
DDDDK

SEQ ID NO: 548 - protein, 4 aa, Artificial
  Xa cleavage site
  MISC_FEATURE (2)..(2): X at position 2 is G or D
IXGR

SEQ ID NO: 549 - protein, 6 aa, Artificial
  Genenase I cleavage site
PGAAHY